European Patent Specification EP 3 187 508 B1, published April 22, 2026. Title: Lysosomal Targeting Peptides and Uses Thereof. Applicant: ZyStor Therapeutics, Inc. The sequence listing filed with the application follows.

SEQUENCE LISTING (35 sequences)

SEQ ID NO: 1 - protein, 67 aa, Homo sapiens
AYRPSETLCGGELVDTLQFVCGDRGFYFSRPASRVSRRSRGIVEECCFRSCDLALLETYCATPAKSE

SEQ ID NO: 2 - protein, 4 aa, Artificial Sequence
  Furin protease recognition sequence
  misc_feature (2)..(3): Xaa can be any naturally occurring amino acid
RXXR

SEQ ID NO: 3 - protein, 6 aa, Artificial Sequence
  Furin protease recognition sequence
  MISC_FEATURE (1)..(1): Xaa is Lys or Arg
  misc_feature (2)..(4): Xaa can be any naturally occurring amino acid
  MISC_FEATURE (5)..(5): Xaa is Lys or Arg
XXXXXR

SEQ ID NO: 4 - protein, 3 aa, Artificial Sequence
  synthetic linker sequence
GAP

SEQ ID NO: 5 - protein, 6 aa, Artificial Sequence
  synthetic linker sequence
GGGGGP

SEQ ID NO: 6 - protein, 8 aa, Artificial Sequence
  Furin cleavage site - p1463 A40
RVSRRSAG

SEQ ID NO: 7 - protein, 3 aa, Artificial Sequence
  synthetic linker sequence
  misc_feature (2)..(2): Xaa can be any naturally occurring amino acid
  MISC_FEATURE (3)..(3): Xaa is Thr or Ser
NXX

SEQ ID NO: 8 - protein, 948 aa, Artificial Sequence
  synthetic ZC-701 construct
AALCGGELVDTLQFVCGDRGFYFSRPASRVSRRSRGIVEECCFRSCDLALLETYCATPAKSEGAPAHPGRPRAVPTQCDVPPNSRFDCAPDKAITQEQCEARGCCYIPAKQGLQGAQMGQPWCFFPPSYPSYKLENLSSSEMGYTATLTRTTPTFFPKDILTLRLDVMMETENRLHFTIKDPANRRYEVPLETPRVHSRAPSPLYSVEFSEEPFGVIVHRQLDGRVLLNTTVAPLFFADQFLQLSTSLPSQYITGLAEHLSPLMLSTSWTRITLWNRDLAPTPGANLYGSHPFYLALEDGGSAHGVFLLNSNAMDVVLQPSPALSWRSTGGILDVYIFLGPEPKSVVQQYLDVVGYPFMPPYWGLGFHLCRWGYSSTAITRQVVENMTRAHFPLDVQWNDLDYMDSRRDFTFNKDGFRDFPAMVQELHQGGRRYMMIVDPAISSSGPAGSYRPYDEGLRRGVFITNETGQPLIGKVWPGSTAFPDFTNPTALAWWEDMVAEFHDQVPFDGMWIDMNEPSNFIRGSEDGCPNNELENPPYVPGVVGGTLQAATICASSHQFLSTHYNLHNLYGLTEAIASHRALVKARGTRPFVISRSTFAGHGRYAGHWTGDVWSSWEQLASSVPEILQFNLLGVPLVGADVCGFLGNTSEELCVRWTQLGAFYPFMRNHNSLLSLPQEPYSFSEPAQQAMRKALTLRYALLPHLYTLFHQAHVAGETVARPLFLEFPKDSSTWTVDHQLLWGEALLITPVLQAGKAEVTGYFPLGTWYDLQTVPIEALGSLPPPPAAPREPAIHSEGQWVTLPAPLDTINVHLRAGYIIPLQGPGLTTTESRQQPMALAVALTKGGEARGELFWDDGESLEVLERGAYTQVIFLARNNTIVNELVRVTSEGAGLQLQKVTVLGVATAPQQVLSNGVPVSNFTYSPDTKVLDICVSLLMGEQFLVSWC

SEQ ID NO: 9 - protein, 4 aa, Artificial Sequence
  sequence proximal to ZC-701 cleavage site
RRSR

SEQ ID NO: 10 - protein, 4 aa, Artificial Sequence
  Furin protease recognition sequence
  misc_feature (2)..(3): Xaa can be any naturally occurring amino acid
RXXR

SEQ ID NO: 11 - DNA, 2970 bp, Artificial Sequence
  GILTd2-7-GAA70-952 cassette
ggtaccagctgctagcaagctaattcacaccaatgggaatcccaatggggaagtcgatgctggtgcttctcaccttcttggccttcgcctcgtgctgcattgctgctctgtgcggcggggagctggtggacaccctccagttcgtctgtggggaccgcggcttctacttcagcaggcccgcaagccgtgtgagccgtcgcagccgtggcatcgttgaggagtgctgtttccgcagctgtgacctggccctcctggagacgtactgtgctacccccgccaagtccgagggcgcgccggcacaccccggccgtcccagagcagtgcccacacagtgcgacgtcccccccaacagccgcttcgattgcgcccctgacaaggccatcacccaggaacagtgcgaggcccgcggctgctgctacatccctgcaaagcaggggctgcagggagcccagatggggcagccctggtgcttcttcccacccagctaccccagctacaagctggagaacctgagctcctctgaaatgggctacacggccaccctgacccgtaccacccccaccttcttccccaaggacatcctgaccctgcggctggacgtgatgatggagactgagaaccgcctccacttcacgatcaaagatccagctaacaggcgctacgaggtgcccttggagaccccgcgtgtccacagccgggcaccgtccccactctacagcgtggagttctctgaggagcccttcggggtgatcgtgcaccggcagctggacggccgcgtgctgctgaacacgacggtggcgcccctgttctttgcggaccagttccttcagctgtccacctcgctgccctcgcagtatatcacaggcctcgccgagcacctcagtcccctgatgctcagcaccagctggaccaggatcaccctgtggaaccgggaccttgcgcccacgcccggtgcgaacctctacgggtctcaccctttctacctggcgctggaggacggcgggtcggcacacggggtgttcctgctaaacagcaatgccatggatgtggtcctgcagccgagccctgcccttagctggaggtcgacaggtgggatcctggatgtctacatcttcctgggcccagagcccaagagcgtggtgcagcagtacctggacgttgtgggatacccgttcatgccgccatactggggcctgggcttccacctgtgccgctggggctactcctccaccgctatcacccgccaggtggtggagaacatgaccagggcccacttccccctggacgtccaatggaacgacctggactacatggactcccggagggacttcacgttcaacaaggatggcttccgggacttcccggccatggtgcaggagctgcaccagggcggccggcgctacatgatgatcgtggatcctgccatcagcagctcgggccctgccgggagctacaggccctacgacgagggtctgcggaggggggttttcatcaccaacgagaccggccagccgctgattgggaaggtatggcccgggtccactgccttccccgacttcaccaaccccacagccctggcctggtgggaggacatggtggctgagttccatgaccaggtgcccttcgacggcatgtggattgacatgaacgagccttccaacttcatcaggggctctgaggacggctgccccaacaatgagctggagaacccaccctacgtgcctggggtggttggggggaccctccaggcggcaaccatctgtgcctccagccaccagtttctctccacacactacaacctgcacaacctctacggcctgaccgaagccatcgcctcccacagggcgctggtgaaggctcgggggacacgcccatttgtgatctcccgctcgacctttgctggccacggccgatacgccggccactggacgggggacgtgtggagctcctgggagcagctcgcctcctccgtgccagaaatcctgcagtttaacctgctgggggtgcctctggtcggggccgacgtctgcggcttcctgggcaacacctcagaggagctgtgtgtgcgctggacccagctgggggccttctaccccttcatgcggaaccacaacagcctgctcagtctgccccaggagccgtacagcttcagcgagccggcccagcaggccatgaggaaggccctcaccctgcgctacgcactcctcccccacctctacacgctgttccaccaggcccacgtcgcgggggagaccgtggcccggcccctcttcctggagttccccaaggactctagcacctggactgtggaccaccagctcctgtggggggaggccctgctcatcaccccagtgctccaggccgggaaggccgaagtgactggctacttccccttgggcacatggtacgacctgcagacggtgccaatagaggcccttggcagcctcccacccccacctgcagctccccgtgagccagccatccacagcgaggggcagtgggtgacgctgccggcccccctggacaccatcaacgtccacctccgggctgggtacatcatccccctgcagggccctggcctcacaaccacagagtcccgccagcagcccatggccctggctgtggccctgaccaagggtggagaggcccgaggggagctgttctgggacgatggagagagcctggaagtgctggagcgaggggcctacacacaggtcatcttcctggccaggaataacacgatcgtgaatgagctggtacgtgtgaccagtgagggagctggcctgcagctgcagaaggtgactgtcctgggcgtggccacggcgccccagcaggtcctctccaacggtgtccctgtctccaacttcacctacagccccgacaccaaggtcctggacatctgtgtctcgctgttgatgggagagcagtttctcgtcagctggtgttagtctagagcttgctagcggccgc

SEQ ID NO: 12 - DNA, 2970 bp, Artificial Sequence
  GILTd2-7/K37-GAA70-952 cassette
ggtaccagctgctagcaagctaattcacaccaatgggaatcccaatggggaagtcgatgctggtgcttctcaccttcttggccttcgcctcgtgctgcattgctgctctgtgcggcggggagctggtggacaccctccagttcgtctgtggggaccgcggcttctacttcagcaggcccgcaagccgtgtgagcaagcgcagccgtggcatcgttgaggagtgctgtttccgcagctgtgacctggccctcctggagacgtactgtgctacccccgccaagtccgagggcgcgccggcacaccccggccgtcccagagcagtgcccacacagtgcgacgtcccccccaacagccgcttcgattgcgcccctgacaaggccatcacccaggaacagtgcgaggcccgcggctgctgctacatccctgcaaagcaggggctgcagggagcccagatggggcagccctggtgcttcttcccacccagctaccccagctacaagctggagaacctgagctcctctgaaatgggctacacggccaccctgacccgtaccacccccaccttcttccccaaggacatcctgaccctgcggctggacgtgatgatggagactgagaaccgcctccacttcacgatcaaagatccagctaacaggcgctacgaggtgcccttggagaccccgcgtgtccacagccgggcaccgtccccactctacagcgtggagttctctgaggagcccttcggggtgatcgtgcaccggcagctggacggccgcgtgctgctgaacacgacggtggcgcccctgttctttgcggaccagttccttcagctgtccacctcgctgccctcgcagtatatcacaggcctcgccgagcacctcagtcccctgatgctcagcaccagctggaccaggatcaccctgtggaaccgggaccttgcgcccacgcccggtgcgaacctctacgggtctcaccctttctacctggcgctggaggacggcgggtcggcacacggggtgttcctgctaaacagcaatgccatggatgtggtcctgcagccgagccctgcccttagctggaggtcgacaggtgggatcctggatgtctacatcttcctgggcccagagcccaagagcgtggtgcagcagtacctggacgttgtgggatacccgttcatgccgccatactggggcctgggcttccacctgtgccgctggggctactcctccaccgctatcacccgccaggtggtggagaacatgaccagggcccacttccccctggacgtccaatggaacgacctggactacatggactcccggagggacttcacgttcaacaaggatggcttccgggacttcccggccatggtgcaggagctgcaccagggcggccggcgctacatgatgatcgtggatcctgccatcagcagctcgggccctgccgggagctacaggccctacgacgagggtctgcggaggggggttttcatcaccaacgagaccggccagccgctgattgggaaggtatggcccgggtccactgccttccccgacttcaccaaccccacagccctggcctggtgggaggacatggtggctgagttccatgaccaggtgcccttcgacggcatgtggattgacatgaacgagccttccaacttcatcaggggctctgaggacggctgccccaacaatgagctggagaacccaccctacgtgcctggggtggttggggggaccctccaggcggcaaccatctgtgcctccagccaccagtttctctccacacactacaacctgcacaacctctacggcctgaccgaagccatcgcctcccacagggcgctggtgaaggctcgggggacacgcccatttgtgatctcccgctcgacctttgctggccacggccgatacgccggccactggacgggggacgtgtggagctcctgggagcagctcgcctcctccgtgccagaaatcctgcagtttaacctgctgggggtgcctctggtcggggccgacgtctgcggcttcctgggcaacacctcagaggagctgtgtgtgcgctggacccagctgggggccttctaccccttcatgcggaaccacaacagcctgctcagtctgccccaggagccgtacagcttcagcgagccggcccagcaggccatgaggaaggccctcaccctgcgctacgcactcctcccccacctctacacgctgttccaccaggcccacgtcgcgggggagaccgtggcccggcccctcttcctggagttccccaaggactctagcacctggactgtggaccaccagctcctgtggggggaggccctgctcatcaccccagtgctccaggccgggaaggccgaagtgactggctacttccccttgggcacatggtacgacctgcagacggtgccaatagaggcccttggcagcctcccacccccacctgcagctccccgtgagccagccatccacagcgaggggcagtgggtgacgctgccggcccccctggacaccatcaacgtccacctccgggctgggtacatcatccccctgcagggccctggcctcacaaccacagagtcccgccagcagcccatggccctggctgtggccctgaccaagggtggagaggcccgaggggagctgttctgggacgatggagagagcctggaagtgctggagcgaggggcctacacacaggtcatcttcctggccaggaataacacgatcgtgaatgagctggtacgtgtgaccagtgagggagctggcctgcagctgcagaaggtgactgtcctgggcgtggccacggcgccccagcaggtcctctccaacggtgtccctgtctccaacttcacctacagccccgacaccaaggtcctggacatctgtgtctcgctgttgatgggagagcagtttctcgtcagctggtgttagtctagagcttgctagcggccgc

SEQ ID NO: 13 - DNA, 2970 bp, Artificial Sequence
  GILTd2-7/K40-GAA70-952 cassette
ggtaccagctgctagcaagctaattcacaccaatgggaatcccaatggggaagtcgatgctggtgcttctcaccttcttggccttcgcctcgtgctgcattgctgctctgtgcggcggggagctggtggacaccctccagttcgtctgtggggaccgcggcttctacttcagcaggcccgcaagccgtgtgagccgtcgcagcaagggcatcgttgaggagtgctgtttccgcagctgtgacctggccctcctggagacgtactgtgctacccccgccaagtccgagggcgcgccggcacaccccggccgtcccagagcagtgcccacacagtgcgacgtcccccccaacagccgcttcgattgcgcccctgacaaggccatcacccaggaacagtgcgaggcccgcggctgctgctacatccctgcaaagcaggggctgcagggagcccagatggggcagccctggtgcttcttcccacccagctaccccagctacaagctggagaacctgagctcctctgaaatgggctacacggccaccctgacccgtaccacccccaccttcttccccaaggacatcctgaccctgcggctggacgtgatgatggagactgagaaccgcctccacttcacgatcaaagatccagctaacaggcgctacgaggtgcccttggagaccccgcgtgtccacagccgggcaccgtccccactctacagcgtggagttctctgaggagcccttcggggtgatcgtgcaccggcagctggacggccgcgtgctgctgaacacgacggtggcgcccctgttctttgcggaccagttccttcagctgtccacctcgctgccctcgcagtatatcacaggcctcgccgagcacctcagtcccctgatgctcagcaccagctggaccaggatcaccctgtggaaccgggaccttgcgcccacgcccggtgcgaacctctacgggtctcaccctttctacctggcgctggaggacggcgggtcggcacacggggtgttcctgctaaacagcaatgccatggatgtggtcctgcagccgagccctgcccttagctggaggtcgacaggtgggatcctggatgtctacatcttcctgggcccagagcccaagagcgtggtgcagcagtacctggacgttgtgggatacccgttcatgccgccatactggggcctgggcttccacctgtgccgctggggctactcctccaccgctatcacccgccaggtggtggagaacatgaccagggcccacttccccctggacgtccaatggaacgacctggactacatggactcccggagggacttcacgttcaacaaggatggcttccgggacttcccggccatggtgcaggagctgcaccagggcggccggcgctacatgatgatcgtggatcctgccatcagcagctcgggccctgccgggagctacaggccctacgacgagggtctgcggaggggggttttcatcaccaacgagaccggccagccgctgattgggaaggtatggcccgggtccactgccttccccgacttcaccaaccccacagccctggcctggtgggaggacatggtggctgagttccatgaccaggtgcccttcgacggcatgtggattgacatgaacgagccttccaacttcatcaggggctctgaggacggctgccccaacaatgagctggagaacccaccctacgtgcctggggtggttggggggaccctccaggcggcaaccatctgtgcctccagccaccagtttctctccacacactacaacctgcacaacctctacggcctgaccgaagccatcgcctcccacagggcgctggtgaaggctcgggggacacgcccatttgtgatctcccgctcgacctttgctggccacggccgatacgccggccactggacgggggacgtgtggagctcctgggagcagctcgcctcctccgtgccagaaatcctgcagtttaacctgctgggggtgcctctggtcggggccgacgtctgcggcttcctgggcaacacctcagaggagctgtgtgtgcgctggacccagctgggggccttctaccccttcatgcggaaccacaacagcctgctcagtctgccccaggagccgtacagcttcagcgagccggcccagcaggccatgaggaaggccctcaccctgcgctacgcactcctcccccacctctacacgctgttccaccaggcccacgtcgcgggggagaccgtggcccggcccctcttcctggagttccccaaggactctagcacctggactgtggaccaccagctcctgtggggggaggccctgctcatcaccccagtgctccaggccgggaaggccgaagtgactggctacttccccttgggcacatggtacgacctgcagacggtgccaatagaggcccttggcagcctcccacccccacctgcagctccccgtgagccagccatccacagcgaggggcagtgggtgacgctgccggcccccctggacaccatcaacgtccacctccgggctgggtacatcatccccctgcagggccctggcctcacaaccacagagtcccgccagcagcccatggccctggctgtggccctgaccaagggtggagaggcccgaggggagctgttctgggacgatggagagagcctggaagtgctggagcgaggggcctacacacaggtcatcttcctggccaggaataacacgatcgtgaatgagctggtacgtgtgaccagtgagggagctggcctgcagctgcagaaggtgactgtcctgggcgtggccacggcgccccagcaggtcctctccaacggtgtccctgtctccaacttcacctacagccccgacaccaaggtcctggacatctgtgtctcgctgttgatgggagagcagtttctcgtcagctggtgttagtctagagcttgctagcggccgc

SEQ ID NO: 14 - DNA, 2970 bp, Artificial Sequence
  GILTd2-7/A37-GAA70-952 cassette
ggtaccagctgctagcaagctaattcacaccaatgggaatcccaatggggaagtcgatgctggtgcttctcaccttcttggccttcgcctcgtgctgcattgctgctctgtgcggcggggagctggtggacaccctccagttcgtctgtggggaccgcggcttctacttcagcaggcccgcaagccgtgtgagcgctcgcagccgtggcatcgttgaggagtgctgtttccgcagctgtgacctggccctcctggagacgtactgtgctacccccgccaagtccgagggcgcgccggcacaccccggccgtcccagagcagtgcccacacagtgcgacgtcccccccaacagccgcttcgattgcgcccctgacaaggccatcacccaggaacagtgcgaggcccgcggctgctgctacatccctgcaaagcaggggctgcagggagcccagatggggcagccctggtgcttcttcccacccagctaccccagctacaagctggagaacctgagctcctctgaaatgggctacacggccaccctgacccgtaccacccccaccttcttccccaaggacatcctgaccctgcggctggacgtgatgatggagactgagaaccgcctccacttcacgatcaaagatccagctaacaggcgctacgaggtgcccttggagaccccgcgtgtccacagccgggcaccgtccccactctacagcgtggagttctctgaggagcccttcggggtgatcgtgcaccggcagctggacggccgcgtgctgctgaacacgacggtggcgcccctgttctttgcggaccagttccttcagctgtccacctcgctgccctcgcagtatatcacaggcctcgccgagcacctcagtcccctgatgctcagcaccagctggaccaggatcaccctgtggaaccgggaccttgcgcccacgcccggtgcgaacctctacgggtctcaccctttctacctggcgctggaggacggcgggtcggcacacggggtgttcctgctaaacagcaatgccatggatgtggtcctgcagccgagccctgcccttagctggaggtcgacaggtgggatcctggatgtctacatcttcctgggcccagagcccaagagcgtggtgcagcagtacctggacgttgtgggatacccgttcatgccgccatactggggcctgggcttccacctgtgccgctggggctactcctccaccgctatcacccgccaggtggtggagaacatgaccagggcccacttccccctggacgtccaatggaacgacctggactacatggactcccggagggacttcacgttcaacaaggatggcttccgggacttcccggccatggtgcaggagctgcaccagggcggccggcgctacatgatgatcgtggatcctgccatcagcagctcgggccctgccgggagctacaggccctacgacgagggtctgcggaggggggttttcatcaccaacgagaccggccagccgctgattgggaaggtatggcccgggtccactgccttccccgacttcaccaaccccacagccctggcctggtgggaggacatggtggctgagttccatgaccaggtgcccttcgacggcatgtggattgacatgaacgagccttccaacttcatcaggggctctgaggacggctgccccaacaatgagctggagaacccaccctacgtgcctggggtggttggggggaccctccaggcggcaaccatctgtgcctccagccaccagtttctctccacacactacaacctgcacaacctctacggcctgaccgaagccatcgcctcccacagggcgctggtgaaggctcgggggacacgcccatttgtgatctcccgctcgacctttgctggccacggccgatacgccggccactggacgggggacgtgtggagctcctgggagcagctcgcctcctccgtgccagaaatcctgcagtttaacctgctgggggtgcctctggtcggggccgacgtctgcggcttcctgggcaacacctcagaggagctgtgtgtgcgctggacccagctgggggccttctaccccttcatgcggaaccacaacagcctgctcagtctgccccaggagccgtacagcttcagcgagccggcccagcaggccatgaggaaggccctcaccctgcgctacgcactcctcccccacctctacacgctgttccaccaggcccacgtcgcgggggagaccgtggcccggcccctcttcctggagttccccaaggactctagcacctggactgtggaccaccagctcctgtggggggaggccctgctcatcaccccagtgctccaggccgggaaggccgaagtgactggctacttccccttgggcacatggtacgacctgcagacggtgccaatagaggcccttggcagcctcccacccccacctgcagctccccgtgagccagccatccacagcgaggggcagtgggtgacgctgccggcccccctggacaccatcaacgtccacctccgggctgggtacatcatccccctgcagggccctggcctcacaaccacagagtcccgccagcagcccatggccctggctgtggccctgaccaagggtggagaggcccgaggggagctgttctgggacgatggagagagcctggaagtgctggagcgaggggcctacacacaggtcatcttcctggccaggaataacacgatcgtgaatgagctggtacgtgtgaccagtgagggagctggcctgcagctgcagaaggtgactgtcctgggcgtggccacggcgccccagcaggtcctctccaacggtgtccctgtctccaacttcacctacagccccgacaccaaggtcctggacatctgtgtctcgctgttgatgggagagcagtttctcgtcagctggtgttagtctagagcttgctagcggccgc

SEQ ID NO: 15 - DNA, 2970 bp, Artificial Sequence
  GILTd2-7/A40-GAA70-952 cassette
ggtaccagctgctagcaagctaattcacaccaatgggaatcccaatggggaagtcgatgctggtgcttctcaccttcttggccttcgcctcgtgctgcattgctgctctgtgcggcggggagctggtggacaccctccagttcgtctgtggggaccgcggcttctacttcagcaggcccgcaagccgtgtgagccgtcgcagcgctggcatcgttgaggagtgctgtttccgcagctgtgacctggccctcctggagacgtactgtgctacccccgccaagtccgagggcgcgccggcacaccccggccgtcccagagcagtgcccacacagtgcgacgtcccccccaacagccgcttcgattgcgcccctgacaaggccatcacccaggaacagtgcgaggcccgcggctgctgctacatccctgcaaagcaggggctgcagggagcccagatggggcagccctggtgcttcttcccacccagctaccccagctacaagctggagaacctgagctcctctgaaatgggctacacggccaccctgacccgtaccacccccaccttcttccccaaggacatcctgaccctgcggctggacgtgatgatggagactgagaaccgcctccacttcacgatcaaagatccagctaacaggcgctacgaggtgcccttggagaccccgcgtgtccacagccgggcaccgtccccactctacagcgtggagttctctgaggagcccttcggggtgatcgtgcaccggcagctggacggccgcgtgctgctgaacacgacggtggcgcccctgttctttgcggaccagttccttcagctgtccacctcgctgccctcgcagtatatcacaggcctcgccgagcacctcagtcccctgatgctcagcaccagctggaccaggatcaccctgtggaaccgggaccttgcgcccacgcccggtgcgaacctctacgggtctcaccctttctacctggcgctggaggacggcgggtcggcacacggggtgttcctgctaaacagcaatgccatggatgtggtcctgcagccgagccctgcccttagctggaggtcgacaggtgggatcctggatgtctacatcttcctgggcccagagcccaagagcgtggtgcagcagtacctggacgttgtgggatacccgttcatgccgccatactggggcctgggcttccacctgtgccgctggggctactcctccaccgctatcacccgccaggtggtggagaacatgaccagggcccacttccccctggacgtccaatggaacgacctggactacatggactcccggagggacttcacgttcaacaaggatggcttccgggacttcccggccatggtgcaggagctgcaccagggcggccggcgctacatgatgatcgtggatcctgccatcagcagctcgggccctgccgggagctacaggccctacgacgagggtctgcggaggggggttttcatcaccaacgagaccggccagccgctgattgggaaggtatggcccgggtccactgccttccccgacttcaccaaccccacagccctggcctggtgggaggacatggtggctgagttccatgaccaggtgcccttcgacggcatgtggattgacatgaacgagccttccaacttcatcaggggctctgaggacggctgccccaacaatgagctggagaacccaccctacgtgcctggggtggttggggggaccctccaggcggcaaccatctgtgcctccagccaccagtttctctccacacactacaacctgcacaacctctacggcctgaccgaagccatcgcctcccacagggcgctggtgaaggctcgggggacacgcccatttgtgatctcccgctcgacctttgctggccacggccgatacgccggccactggacgggggacgtgtggagctcctgggagcagctcgcctcctccgtgccagaaatcctgcagtttaacctgctgggggtgcctctggtcggggccgacgtctgcggcttcctgggcaacacctcagaggagctgtgtgtgcgctggacccagctgggggccttctaccccttcatgcggaaccacaacagcctgctcagtctgccccaggagccgtacagcttcagcgagccggcccagcaggccatgaggaaggccctcaccctgcgctacgcactcctcccccacctctacacgctgttccaccaggcccacgtcgcgggggagaccgtggcccggcccctcttcctggagttccccaaggactctagcacctggactgtggaccaccagctcctgtggggggaggccctgctcatcaccccagtgctccaggccgggaaggccgaagtgactggctacttccccttgggcacatggtacgacctgcagacggtgccaatagaggcccttggcagcctcccacccccacctgcagctccccgtgagccagccatccacagcgaggggcagtgggtgacgctgccggcccccctggacaccatcaacgtccacctccgggctgggtacatcatccccctgcagggccctggcctcacaaccacagagtcccgccagcagcccatggccctggctgtggccctgaccaagggtggagaggcccgaggggagctgttctgggacgatggagagagcctggaagtgctggagcgaggggcctacacacaggtcatcttcctggccaggaataacacgatcgtgaatgagctggtacgtgtgaccagtgagggagctggcctgcagctgcagaaggtgactgtcctgggcgtggccacggcgccccagcaggtcctctccaacggtgtccctgtctccaacttcacctacagccccgacaccaaggtcctggacatctgtgtctcgctgttgatgggagagcagtttctcgtcagctggtgttagtctagagcttgctagcggccgc

SEQ ID NO: 16 - DNA, 2953 bp, Artificial Sequence
  GILTd2-7M1/K37-GAA70-952 cassette
ggtaccaagcttgccatgggaatcccaatgggcaagtcgatgctggtgctgctcaccttcttggcctttgcctcgtgctgcattgccgctctgtgcggcggggaactggtggacaccctccaattcgtctgtggggaccggggcttctacttcagcagacccgcaagccgtgtgagtaagcgcagccgtggcattgttgaggagtgctgttttcgcagctgtgacctggctctcctggagacgtactgcgctacccccgccaagtctgagggcgcgccggcacaccccggccgtcccagagcagtgcccacacagtgcgacgtcccccccaacagccgcttcgattgcgcccctgacaaggccatcacccaggaacagtgcgaggcccgcggctgctgctacatccctgcaaagcaggggctgcagggagcccagatggggcagccctggtgcttcttcccacccagctaccccagctacaagctggagaacctgagctcctctgaaatgggctacacggccaccctgacccgtaccacccccaccttcttccccaaggacatcctgaccctgcggctggacgtgatgatggagactgagaaccgcctccacttcacgatcaaagatccagctaacaggcgctacgaggtgcccttggagaccccgcgtgtccacagccgggcaccgtccccactctacagcgtggagttctctgaggagcccttcggggtgatcgtgcaccggcagctggacggccgcgtgctgctgaacacgacggtggcgcccctgttctttgcggaccagttccttcagctgtccacctcgctgccctcgcagtatatcacaggcctcgccgagcacctcagtcccctgatgctcagcaccagctggaccaggatcaccctgtggaaccgggaccttgcgcccacgcccggtgcgaacctctacgggtctcaccctttctacctggcgctggaggacggcgggtcggcacacggggtgttcctgctaaacagcaatgccatggatgtggtcctgcagccgagccctgcccttagctggaggtcgacaggtgggatcctggatgtctacatcttcctgggcccagagcccaagagcgtggtgcagcagtacctggacgttgtgggatacccgttcatgccgccatactggggcctgggcttccacctgtgccgctggggctactcctccaccgctatcacccgccaggtggtggagaacatgaccagggcccacttccccctggacgtccaatggaacgacctggactacatggactcccggagggacttcacgttcaacaaggatggcttccgggacttcccggccatggtgcaggagctgcaccagggcggccggcgctacatgatgatcgtggatcctgccatcagcagctcgggccctgccgggagctacaggccctacgacgagggtctgcggaggggggttttcatcaccaacgagaccggccagccgctgattgggaaggtatggcccgggtccactgccttccccgacttcaccaaccccacagccctggcctggtgggaggacatggtggctgagttccatgaccaggtgcccttcgacggcatgtggattgacatgaacgagccttccaacttcatcaggggctctgaggacggctgccccaacaatgagctggagaacccaccctacgtgcctggggtggttggggggaccctccaggcggcaaccatctgtgcctccagccaccagtttctctccacacactacaacctgcacaacctctacggcctgaccgaagccatcgcctcccacagggcgctggtgaaggctcgggggacacgcccatttgtgatctcccgctcgacctttgctggccacggccgatacgccggccactggacgggggacgtgtggagctcctgggagcagctcgcctcctccgtgccagaaatcctgcagtttaacctgctgggggtgcctctggtcggggccgacgtctgcggcttcctgggcaacacctcagaggagctgtgtgtgcgctggacccagctgggggccttctaccccttcatgcggaaccacaacagcctgctcagtctgccccaggagccgtacagcttcagcgagccggcccagcaggccatgaggaaggccctcaccctgcgctacgcactcctcccccacctctacacgctgttccaccaggcccacgtcgcgggggagaccgtggcccggcccctcttcctggagttccccaaggactctagcacctggactgtggaccaccagctcctgtggggggaggccctgctcatcaccccagtgctccaggccgggaaggccgaagtgactggctacttccccttgggcacatggtacgacctgcagacggtgccaatagaggcccttggcagcctcccacccccacctgcagctccccgtgagccagccatccacagcgaggggcagtgggtgacgctgccggcccccctggacaccatcaacgtccacctccgggctgggtacatcatccccctgcagggccctggcctcacaaccacagagtcccgccagcagcccatggccctggctgtggccctgaccaagggtggagaggcccgaggggagctgttctgggacgatggagagagcctggaagtgctggagcgaggggcctacacacaggtcatcttcctggccaggaataacacgatcgtgaatgagctggtacgtgtgaccagtgagggagctggcctgcagctgcagaaggtgactgtcctgggcgtggccacggcgccccagcaggtcctctccaacggtgtccctgtctccaacttcacctacagccccgacaccaaggtcctggacatctgtgtctcgctgttgatgggagagcagtttctcgtcagctggtgttagtctagagcttgctagcggccgc

SEQ ID NO: 17 - DNA, 2953 bp, Artificial Sequence
  GILTd2-7M1/A37-GAA70-952 cassette
ggtaccaagcttgccatgggaatcccaatgggcaagtcgatgctggtgctgctcaccttcttggcctttgcctcgtgctgcattgccgctctgtgcggcggggaactggtggacaccctccaattcgtctgtggggaccggggcttctacttcagcagacccgcaagccgtgtgagtgctcgcagccgtggcattgttgaggagtgctgttttcgcagctgtgacctggctctcctggagacgtactgcgctacccccgccaagtctgagggcgcgccggcacaccccggccgtcccagagcagtgcccacacagtgcgacgtcccccccaacagccgcttcgattgcgcccctgacaaggccatcacccaggaacagtgcgaggcccgcggctgctgctacatccctgcaaagcaggggctgcagggagcccagatggggcagccctggtgcttcttcccacccagctaccccagctacaagctggagaacctgagctcctctgaaatgggctacacggccaccctgacccgtaccacccccaccttcttccccaaggacatcctgaccctgcggctggacgtgatgatggagactgagaaccgcctccacttcacgatcaaagatccagctaacaggcgctacgaggtgcccttggagaccccgcgtgtccacagccgggcaccgtccccactctacagcgtggagttctctgaggagcccttcggggtgatcgtgcaccggcagctggacggccgcgtgctgctgaacacgacggtggcgcccctgttctttgcggaccagttccttcagctgtccacctcgctgccctcgcagtatatcacaggcctcgccgagcacctcagtcccctgatgctcagcaccagctggaccaggatcaccctgtggaaccgggaccttgcgcccacgcccggtgcgaacctctacgggtctcaccctttctacctggcgctggaggacggcgggtcggcacacggggtgttcctgctaaacagcaatgccatggatgtggtcctgcagccgagccctgcccttagctggaggtcgacaggtgggatcctggatgtctacatcttcctgggcccagagcccaagagcgtggtgcagcagtacctggacgttgtgggatacccgttcatgccgccatactggggcctgggcttccacctgtgccgctggggctactcctccaccgctatcacccgccaggtggtggagaacatgaccagggcccacttccccctggacgtccaatggaacgacctggactacatggactcccggagggacttcacgttcaacaaggatggcttccgggacttcccggccatggtgcaggagctgcaccagggcggccggcgctacatgatgatcgtggatcctgccatcagcagctcgggccctgccgggagctacaggccctacgacgagggtctgcggaggggggttttcatcaccaacgagaccggccagccgctgattgggaaggtatggcccgggtccactgccttccccgacttcaccaaccccacagccctggcctggtgggaggacatggtggctgagttccatgaccaggtgcccttcgacggcatgtggattgacatgaacgagccttccaacttcatcaggggctctgaggacggctgccccaacaatgagctggagaacccaccctacgtgcctggggtggttggggggaccctccaggcggcaaccatctgtgcctccagccaccagtttctctccacacactacaacctgcacaacctctacggcctgaccgaagccatcgcctcccacagggcgctggtgaaggctcgggggacacgcccatttgtgatctcccgctcgacctttgctggccacggccgatacgccggccactggacgggggacgtgtggagctcctgggagcagctcgcctcctccgtgccagaaatcctgcagtttaacctgctgggggtgcctctggtcggggccgacgtctgcggcttcctgggcaacacctcagaggagctgtgtgtgcgctggacccagctgggggccttctaccccttcatgcggaaccacaacagcctgctcagtctgccccaggagccgtacagcttcagcgagccggcccagcaggccatgaggaaggccctcaccctgcgctacgcactcctcccccacctctacacgctgttccaccaggcccacgtcgcgggggagaccgtggcccggcccctcttcctggagttccccaaggactctagcacctggactgtggaccaccagctcctgtggggggaggccctgctcatcaccccagtgctccaggccgggaaggccgaagtgactggctacttccccttgggcacatggtacgacctgcagacggtgccaatagaggcccttggcagcctcccacccccacctgcagctccccgtgagccagccatccacagcgaggggcagtgggtgacgctgccggcccccctggacaccatcaacgtccacctccgggctgggtacatcatccccctgcagggccctggcctcacaaccacagagtcccgccagcagcccatggccctggctgtggccctgaccaagggtggagaggcccgaggggagctgttctgggacgatggagagagcctggaagtgctggagcgaggggcctacacacaggtcatcttcctggccaggaataacacgatcgtgaatgagctggtacgtgtgaccagtgagggagctggcctgcagctgcagaaggtgactgtcctgggcgtggccacggcgccccagcaggtcctctccaacggtgtccctgtctccaacttcacctacagccccgacaccaaggtcctggacatctgtgtctcgctgttgatgggagagcagtttctcgtcagctggtgttagtctagagcttgctagcggccgc

SEQ ID NO: 18 - DNA, 2940 bp, Artificial Sequence
  GILTd2-7d30-39-GAA70-952 cassette
ggtaccagctgctagcaagctaattcacaccaatgggaatcccaatggggaagtcgatgctggtgcttctcaccttcttggccttcgcctcgtgctgcattgctgctctgtgcggcggggagctggtggacaccctccagttcgtctgtggggaccgcggcttctacttcagccgtggcatcgttgaggagtgctgtttccgcagctgtgacctggccctcctggagacgtactgtgctacccccgccaagtccgagggcgcgccggcacaccccggccgtcccagagcagtgcccacacagtgcgacgtcccccccaacagccgcttcgattgcgcccctgacaaggccatcacccaggaacagtgcgaggcccgcggctgctgctacatccctgcaaagcaggggctgcagggagcccagatggggcagccctggtgcttcttcccacccagctaccccagctacaagctggagaacctgagctcctctgaaatgggctacacggccaccctgacccgtaccacccccaccttcttccccaaggacatcctgaccctgcggctggacgtgatgatggagactgagaaccgcctccacttcacgatcaaagatccagctaacaggcgctacgaggtgcccttggagaccccgcgtgtccacagccgggcaccgtccccactctacagcgtggagttctctgaggagcccttcggggtgatcgtgcaccggcagctggacggccgcgtgctgctgaacacgacggtggcgcccctgttctttgcggaccagttccttcagctgtccacctcgctgccctcgcagtatatcacaggcctcgccgagcacctcagtcccctgatgctcagcaccagctggaccaggatcaccctgtggaaccgggaccttgcgcccacgcccggtgcgaacctctacgggtctcaccctttctacctggcgctggaggacggcgggtcggcacacggggtgttcctgctaaacagcaatgccatggatgtggtcctgcagccgagccctgcccttagctggaggtcgacaggtgggatcctggatgtctacatcttcctgggcccagagcccaagagcgtggtgcagcagtacctggacgttgtgggatacccgttcatgccgccatactggggcctgggcttccacctgtgccgctggggctactcctccaccgctatcacccgccaggtggtggagaacatgaccagggcccacttccccctggacgtccaatggaacgacctggactacatggactcccggagggacttcacgttcaacaaggatggcttccgggacttcccggccatggtgcaggagctgcaccagggcggccggcgctacatgatgatcgtggatcctgccatcagcagctcgggccctgccgggagctacaggccctacgacgagggtctgcggaggggggttttcatcaccaacgagaccggccagccgctgattgggaaggtatggcccgggtccactgccttccccgacttcaccaaccccacagccctggcctggtgggaggacatggtggctgagttccatgaccaggtgcccttcgacggcatgtggattgacatgaacgagccttccaacttcatcaggggctctgaggacggctgccccaacaatgagctggagaacccaccctacgtgcctggggtggttggggggaccctccaggcggcaaccatctgtgcctccagccaccagtttctctccacacactacaacctgcacaacctctacggcctgaccgaagccatcgcctcccacagggcgctggtgaaggctcgggggacacgcccatttgtgatctcccgctcgacctttgctggccacggccgatacgccggccactggacgggggacgtgtggagctcctgggagcagctcgcctcctccgtgccagaaatcctgcagtttaacctgctgggggtgcctctggtcggggccgacgtctgcggcttcctgggcaacacctcagaggagctgtgtgtgcgctggacccagctgggggccttctaccccttcatgcggaaccacaacagcctgctcagtctgccccaggagccgtacagcttcagcgagccggcccagcaggccatgaggaaggccctcaccctgcgctacgcactcctcccccacctctacacgctgttccaccaggcccacgtcgcgggggagaccgtggcccggcccctcttcctggagttccccaaggactctagcacctggactgtggaccaccagctcctgtggggggaggccctgctcatcaccccagtgctccaggccgggaaggccgaagtgactggctacttccccttgggcacatggtacgacctgcagacggtgccaatagaggcccttggcagcctcccacccccacctgcagctccccgtgagccagccatccacagcgaggggcagtgggtgacgctgccggcccccctggacaccatcaacgtccacctccgggctgggtacatcatccccctgcagggccctggcctcacaaccacagagtcccgccagcagcccatggccctggctgtggccctgaccaagggtggagaggcccgaggggagctgttctgggacgatggagagagcctggaagtgctggagcgaggggcctacacacaggtcatcttcctggccaggaataacacgatcgtgaatgagctggtacgtgtgaccagtgagggagctggcctgcagctgcagaaggtgactgtcctgggcgtggccacggcgccccagcaggtcctctccaacggtgtccctgtctccaacttcacctacagccccgacaccaaggtcctggacatctgtgtctcgctgttgatgggagagcagtttctcgtcagctggtgttagtctagagcttgctagcggccgc

SEQ ID NO: 19 - DNA, 2943 bp, Artificial Sequence
  GILTd2-7d31-39-GAA70-952 cassette
ggtaccagctgctagcaagctaattcacaccaatgggaatcccaatggggaagtcgatgctggtgcttctcaccttcttggccttcgcctcgtgctgcattgctgctctgtgcggcggggagctggtggacaccctccagttcgtctgtggggaccgcggcttctacttcagcaggcgtggcatcgttgaggagtgctgtttccgcagctgtgacctggccctcctggagacgtactgtgctacccccgccaagtccgagggcgcgccggcacaccccggccgtcccagagcagtgcccacacagtgcgacgtcccccccaacagccgcttcgattgcgcccctgacaaggccatcacccaggaacagtgcgaggcccgcggctgctgctacatccctgcaaagcaggggctgcagggagcccagatggggcagccctggtgcttcttcccacccagctaccccagctacaagctggagaacctgagctcctctgaaatgggctacacggccaccctgacccgtaccacccccaccttcttccccaaggacatcctgaccctgcggctggacgtgatgatggagactgagaaccgcctccacttcacgatcaaagatccagctaacaggcgctacgaggtgcccttggagaccccgcgtgtccacagccgggcaccgtccccactctacagcgtggagttctctgaggagcccttcggggtgatcgtgcaccggcagctggacggccgcgtgctgctgaacacgacggtggcgcccctgttctttgcggaccagttccttcagctgtccacctcgctgccctcgcagtatatcacaggcctcgccgagcacctcagtcccctgatgctcagcaccagctggaccaggatcaccctgtggaaccgggaccttgcgcccacgcccggtgcgaacctctacgggtctcaccctttctacctggcgctggaggacggcgggtcggcacacggggtgttcctgctaaacagcaatgccatggatgtggtcctgcagccgagccctgcccttagctggaggtcgacaggtgggatcctggatgtctacatcttcctgggcccagagcccaagagcgtggtgcagcagtacctggacgttgtgggatacccgttcatgccgccatactggggcctgggcttccacctgtgccgctggggctactcctccaccgctatcacccgccaggtggtggagaacatgaccagggcccacttccccctggacgtccaatggaacgacctggactacatggactcccggagggacttcacgttcaacaaggatggcttccgggacttcccggccatggtgcaggagctgcaccagggcggccggcgctacatgatgatcgtggatcctgccatcagcagctcgggccctgccgggagctacaggccctacgacgagggtctgcggaggggggttttcatcaccaacgagaccggccagccgctgattgggaaggtatggcccgggtccactgccttccccgacttcaccaaccccacagccctggcctggtgggaggacatggtggctgagttccatgaccaggtgcccttcgacggcatgtggattgacatgaacgagccttccaacttcatcaggggctctgaggacggctgccccaacaatgagctggagaacccaccctacgtgcctggggtggttggggggaccctccaggcggcaaccatctgtgcctccagccaccagtttctctccacacactacaacctgcacaacctctacggcctgaccgaagccatcgcctcccacagggcgctggtgaaggctcgggggacacgcccatttgtgatctcccgctcgacctttgctggccacggccgatacgccggccactggacgggggacgtgtggagctcctgggagcagctcgcctcctccgtgccagaaatcctgcagtttaacctgctgggggtgcctctggtcggggccgacgtctgcggcttcctgggcaacacctcagaggagctgtgtgtgcgctggacccagctgggggccttctaccccttcatgcggaaccacaacagcctgctcagtctgccccaggagccgtacagcttcagcgagccggcccagcaggccatgaggaaggccctcaccctgcgctacgcactcctcccccacctctacacgctgttccaccaggcccacgtcgcgggggagaccgtggcccggcccctcttcctggagttccccaaggactctagcacctggactgtggaccaccagctcctgtggggggaggccctgctcatcaccccagtgctccaggccgggaaggccgaagtgactggctacttccccttgggcacatggtacgacctgcagacggtgccaatagaggcccttggcagcctcccacccccacctgcagctccccgtgagccagccatccacagcgaggggcagtgggtgacgctgccggcccccctggacaccatcaacgtccacctccgggctgggtacatcatccccctgcagggccctggcctcacaaccacagagtcccgccagcagcccatggccctggctgtggccctgaccaagggtggagaggcccgaggggagctgttctgggacgatggagagagcctggaagtgctggagcgaggggcctacacacaggtcatcttcctggccaggaataacacgatcgtgaatgagctggtacgtgtgaccagtgagggagctggcctgcagctgcagaaggtgactgtcctgggcgtggccacggcgccccagcaggtcctctccaacggtgtccctgtctccaacttcacctacagccccgacaccaaggtcctggacatctgtgtctcgctgttgatgggagagcagtttctcgtcagctggtgttagtctagagcttgctagcggccgc

SEQ ID NO: 20 - DNA, 2946 bp, Artificial Sequence
  GILTd2-7d32-39-GAA70-952 cassette
ggtaccagctgctagcaagctaattcacaccaatgggaatcccaatggggaagtcgatgctggtgcttctcaccttcttggccttcgcctcgtgctgcattgctgctctgtgcggcggggagctggtggacaccctccagttcgtctgtggggaccgcggcttctacttcagcaggccccgtggcatcgttgaggagtgctgtttccgcagctgtgacctggccctcctggagacgtactgtgctacccccgccaagtccgagggcgcgccggcacaccccggccgtcccagagcagtgcccacacagtgcgacgtcccccccaacagccgcttcgattgcgcccctgacaaggccatcacccaggaacagtgcgaggcccgcggctgctgctacatccctgcaaagcaggggctgcagggagcccagatggggcagccctggtgcttcttcccacccagctaccccagctacaagctggagaacctgagctcctctgaaatgggctacacggccaccctgacccgtaccacccccaccttcttccccaaggacatcctgaccctgcggctggacgtgatgatggagactgagaaccgcctccacttcacgatcaaagatccagctaacaggcgctacgaggtgcccttggagaccccgcgtgtccacagccgggcaccgtccccactctacagcgtggagttctctgaggagcccttcggggtgatcgtgcaccggcagctggacggccgcgtgctgctgaacacgacggtggcgcccctgttctttgcggaccagttccttcagctgtccacctcgctgccctcgcagtatatcacaggcctcgccgagcacctcagtcccctgatgctcagcaccagctggaccaggatcaccctgtggaaccgggaccttgcgcccacgcccggtgcgaacctctacgggtctcaccctttctacctggcgctggaggacggcgggtcggcacacggggtgttcctgctaaacagcaatgccatggatgtggtcctgcagccgagccctgcccttagctggaggtcgacaggtgggatcctggatgtctacatcttcctgggcccagagcccaagagcgtggtgcagcagtacctggacgttgtgggatacccgttcatgccgccatactggggcctgggcttccacctgtgccgctggggctactcctccaccgctatcacccgccaggtggtggagaacatgaccagggcccacttccccctggacgtccaatggaacgacctggactacatggactcccggagggacttcacgttcaacaaggatggcttccgggacttcccggccatggtgcaggagctgcaccagggcggccggcgctacatgatgatcgtggatcctgccatcagcagctcgggccctgccgggagctacaggccctacgacgagggtctgcggaggggggttttcatcaccaacgagaccggccagccgctgattgggaaggtatggcccgggtccactgccttccccgacttcaccaaccccacagccctggcctggtgggaggacatggtggctgagttccatgaccaggtgcccttcgacggcatgtggattgacatgaacgagccttccaacttcatcaggggctctgaggacggctgccccaacaatgagctggagaacccaccctacgtgcctggggtggttggggggaccctccaggcggcaaccatctgtgcctccagccaccagtttctctccacacactacaacctgcacaacctctacggcctgaccgaagccatcgcctcccacagggcgctggtgaaggctcgggggacacgcccatttgtgatctcccgctcgacctttgctggccacggccgatacgccggccactggacgggggacgtgtggagctcctgggagcagctcgcctcctccgtgccagaaatcctgcagtttaacctgctgggggtgcctctggtcggggccgacgtctgcggcttcctgggcaacacctcagaggagctgtgtgtgcgctggacccagctgggggccttctaccccttcatgcggaaccacaacagcctgctcagtctgccccaggagccgtacagcttcagcgagccggcccagcaggccatgaggaaggccctcaccctgcgctacgcactcctcccccacctctacacgctgttccaccaggcccacgtcgcgggggagaccgtggcccggcccctcttcctggagttccccaaggactctagcacctggactgtggaccaccagctcctgtggggggaggccctgctcatcaccccagtgctccaggccgggaaggccgaagtgactggctacttccccttgggcacatggtacgacctgcagacggtgccaatagaggcccttggcagcctcccacccccacctgcagctccccgtgagccagccatccacagcgaggggcagtgggtgacgctgccggcccccctggacaccatcaacgtccacctccgggctgggtacatcatccccctgcagggccctggcctcacaaccacagagtcccgccagcagcccatggccctggctgtggccctgaccaagggtggagaggcccgaggggagctgttctgggacgatggagagagcctggaagtgctggagcgaggggcctacacacaggtcatcttcctggccaggaataacacgatcgtgaatgagctggtacgtgtgaccagtgagggagctggcctgcagctgcagaaggtgactgtcctgggcgtggccacggcgccccagcaggtcctctccaacggtgtccctgtctccaacttcacctacagccccgacaccaaggtcctggacatctgtgtctcgctgttgatgggagagcagtttctcgtcagctggtgttagtctagagcttgctagcggccgc

SEQ ID NO: 21 - DNA, 2949 bp, Artificial Sequence
  GILTd2-7d33-39-GAA70-952 cassette
ggtaccagctgctagcaagctaattcacaccaatgggaatcccaatggggaagtcgatgctggtgcttctcaccttcttggccttcgcctcgtgctgcattgctgctctgtgcggcggggagctggtggacaccctccagttcgtctgtggggaccgcggcttctacttcagcaggcccgcacgtggcatcgttgaggagtgctgtttccgcagctgtgacctggccctcctggagacgtactgtgctacccccgccaagtccgagggcgcgccggcacaccccggccgtcccagagcagtgcccacacagtgcgacgtcccccccaacagccgcttcgattgcgcccctgacaaggccatcacccaggaacagtgcgaggcccgcggctgctgctacatccctgcaaagcaggggctgcagggagcccagatggggcagccctggtgcttcttcccacccagctaccccagctacaagctggagaacctgagctcctctgaaatgggctacacggccaccctgacccgtaccacccccaccttcttccccaaggacatcctgaccctgcggctggacgtgatgatggagactgagaaccgcctccacttcacgatcaaagatccagctaacaggcgctacgaggtgcccttggagaccccgcgtgtccacagccgggcaccgtccccactctacagcgtggagttctctgaggagcccttcggggtgatcgtgcaccggcagctggacggccgcgtgctgctgaacacgacggtggcgcccctgttctttgcggaccagttccttcagctgtccacctcgctgccctcgcagtatatcacaggcctcgccgagcacctcagtcccctgatgctcagcaccagctggaccaggatcaccctgtggaaccgggaccttgcgcccacgcccggtgcgaacctctacgggtctcaccctttctacctggcgctggaggacggcgggtcggcacacggggtgttcctgctaaacagcaatgccatggatgtggtcctgcagccgagccctgcccttagctggaggtcgacaggtgggatcctggatgtctacatcttcctgggcccagagcccaagagcgtggtgcagcagtacctggacgttgtgggatacccgttcatgccgccatactggggcctgggcttccacctgtgccgctggggctactcctccaccgctatcacccgccaggtggtggagaacatgaccagggcccacttccccctggacgtccaatggaacgacctggactacatggactcccggagggacttcacgttcaacaaggatggcttccgggacttcccggccatggtgcaggagctgcaccagggcggccggcgctacatgatgatcgtggatcctgccatcagcagctcgggccctgccgggagctacaggccctacgacgagggtctgcggaggggggttttcatcaccaacgagaccggccagccgctgattgggaaggtatggcccgggtccactgccttccccgacttcaccaaccccacagccctggcctggtgggaggacatggtggctgagttccatgaccaggtgcccttcgacggcatgtggattgacatgaacgagccttccaacttcatcaggggctctgaggacggctgccccaacaatgagctggagaacccaccctacgtgcctggggtggttggggggaccctccaggcggcaaccatctgtgcctccagccaccagtttctctccacacactacaacctgcacaacctctacggcctgaccgaagccatcgcctcccacagggcgctggtgaaggctcgggggacacgcccatttgtgatctcccgctcgacctttgctggccacggccgatacgccggccactggacgggggacgtgtggagctcctgggagcagctcgcctcctccgtgccagaaatcctgcagtttaacctgctgggggtgcctctggtcggggccgacgtctgcggcttcctgggcaacacctcagaggagctgtgtgtgcgctggacccagctgggggccttctaccccttcatgcggaaccacaacagcctgctcagtctgccccaggagccgtacagcttcagcgagccggcccagcaggccatgaggaaggccctcaccctgcgctacgcactcctcccccacctctacacgctgttccaccaggcccacgtcgcgggggagaccgtggcccggcccctcttcctggagttccccaaggactctagcacctggactgtggaccaccagctcctgtggggggaggccctgctcatcaccccagtgctccaggccgggaaggccgaagtgactggctacttccccttgggcacatggtacgacctgcagacggtgccaatagaggcccttggcagcctcccacccccacctgcagctccccgtgagccagccatccacagcgaggggcagtgggtgacgctgccggcccccctggacaccatcaacgtccacctccgggctgggtacatcatccccctgcagggccctggcctcacaaccacagagtcccgccagcagcccatggccctggctgtggccctgaccaagggtggagaggcccgaggggagctgttctgggacgatggagagagcctggaagtgctggagcgaggggcctacacacaggtcatcttcctggccaggaataacacgatcgtgaatgagctggtacgtgtgaccagtgagggagctggcctgcagctgcagaaggtgactgtcctgggcgtggccacggcgccccagcaggtcctctccaacggtgtccctgtctccaacttcacctacagccccgacaccaaggtcctggacatctgtgtctcgctgttgatgggagagcagtttctcgtcagctggtgttagtctagagcttgctagcggccgc

SEQ ID NO: 22 - DNA, 2952 bp, Artificial Sequence
  GILTd2-7d34-39-GAA70-952 cassette
ggtaccagctgctagcaagctaattcacaccaatgggaatcccaatggggaagtcgatgctggtgcttctcaccttcttggccttcgcctcgtgctgcattgctgctctgtgcggcggggagctggtggacaccctccagttcgtctgtggggaccgcggcttctacttcagcaggcccgcaagccgtggcatcgttgaggagtgctgtttccgcagctgtgacctggccctcctggagacgtactgtgctacccccgccaagtccgagggcgcgccggcacaccccggccgtcccagagcagtgcccacacagtgcgacgtcccccccaacagccgcttcgattgcgcccctgacaaggccatcacccaggaacagtgcgaggcccgcggctgctgctacatccctgcaaagcaggggctgcagggagcccagatggggcagccctggtgcttcttcccacccagctaccccagctacaagctggagaacctgagctcctctgaaatgggctacacggccaccctgacccgtaccacccccaccttcttccccaaggacatcctgaccctgcggctggacgtgatgatggagactgagaaccgcctccacttcacgatcaaagatccagctaacaggcgctacgaggtgcccttggagaccccgcgtgtccacagccgggcaccgtccccactctacagcgtggagttctctgaggagcccttcggggtgatcgtgcaccggcagctggacggccgcgtgctgctgaacacgacggtggcgcccctgttctttgcggaccagttccttcagctgtccacctcgctgccctcgcagtatatcacaggcctcgccgagcacctcagtcccctgatgctcagcaccagctggaccaggatcaccctgtggaaccgggaccttgcgcccacgcccggtgcgaacctctacgggtctcaccctttctacctggcgctggaggacggcgggtcggcacacggggtgttcctgctaaacagcaatgccatggatgtggtcctgcagccgagccctgcccttagctggaggtcgacaggtgggatcctggatgtctacatcttcctgggcccagagcccaagagcgtggtgcagcagtacctggacgttgtgggatacccgttcatgccgccatactggggcctgggcttccacctgtgccgctggggctactcctccaccgctatcacccgccaggtggtggagaacatgaccagggcccacttccccctggacgtccaatggaacgacctggactacatggactcccggagggacttcacgttcaacaaggatggcttccgggacttcccggccatggtgcaggagctgcaccagggcggccggcgctacatgatgatcgtggatcctgccatcagcagctcgggccctgccgggagctacaggccctacgacgagggtctgcggaggggggttttcatcaccaacgagaccggccagccgctgattgggaaggtatggcccgggtccactgccttccccgacttcaccaaccccacagccctggcctggtgggaggacatggtggctgagttccatgaccaggtgcccttcgacggcatgtggattgacatgaacgagccttccaacttcatcaggggctctgaggacggctgccccaacaatgagctggagaacccaccctacgtgcctggggtggttggggggaccctccaggcggcaaccatctgtgcctccagccaccagtttctctccacacactacaacctgcacaacctctacggcctgaccgaagccatcgcctcccacagggcgctggtgaaggctcgggggacacgcccatttgtgatctcccgctcgacctttgctggccacggccgatacgccggccactggacgggggacgtgtggagctcctgggagcagctcgcctcctccgtgccagaaatcctgcagtttaacctgctgggggtgcctctggtcggggccgacgtctgcggcttcctgggcaacacctcagaggagctgtgtgtgcgctggacccagctgggggccttctaccccttcatgcggaaccacaacagcctgctcagtctgccccaggagccgtacagcttcagcgagccggcccagcaggccatgaggaaggccctcaccctgcgctacgcactcctcccccacctctacacgctgttccaccaggcccacgtcgcgggggagaccgtggcccggcccctcttcctggagttccccaaggactctagcacctggactgtggaccaccagctcctgtggggggaggccctgctcatcaccccagtgctccaggccgggaaggccgaagtgactggctacttccccttgggcacatggtacgacctgcagacggtgccaatagaggcccttggcagcctcccacccccacctgcagctccccgtgagccagccatccacagcgaggggcagtgggtgacgctgccggcccccctggacaccatcaacgtccacctccgggctgggtacatcatccccctgcagggccctggcctcacaaccacagagtcccgccagcagcccatggccctggctgtggccctgaccaagggtggagaggcccgaggggagctgttctgggacgatggagagagcctggaagtgctggagcgaggggcctacacacaggtcatcttcctggccaggaataacacgatcgtgaatgagctggtacgtgtgaccagtgagggagctggcctgcagctgcagaaggtgactgtcctgggcgtggccacggcgccccagcaggtcctctccaacggtgtccctgtctccaacttcacctacagccccgacaccaaggtcctggacatctgtgtctcgctgttgatgggagagcagtttctcgtcagctggtgttagtctagagcttgctagcggccgc

SEQ ID NO: 23 - DNA, 2955 bp, Artificial Sequence
  GILTd2-7d35-39-GAA70-952 cassette
ggtaccagctgctagcaagctaattcacaccaatgggaatcccaatggggaagtcgatgctggtgcttctcaccttcttggccttcgcctcgtgctgcattgctgctctgtgcggcggggagctggtggacaccctccagttcgtctgtggggaccgcggcttctacttcagcaggcccgcaagccgtcgtggcatcgttgaggagtgctgtttccgcagctgtgacctggccctcctggagacgtactgtgctacccccgccaagtccgagggcgcgccggcacaccccggccgtcccagagcagtgcccacacagtgcgacgtcccccccaacagccgcttcgattgcgcccctgacaaggccatcacccaggaacagtgcgaggcccgcggctgctgctacatccctgcaaagcaggggctgcagggagcccagatggggcagccctggtgcttcttcccacccagctaccccagctacaagctggagaacctgagctcctctgaaatgggctacacggccaccctgacccgtaccacccccaccttcttccccaaggacatcctgaccctgcggctggacgtgatgatggagactgagaaccgcctccacttcacgatcaaagatccagctaacaggcgctacgaggtgcccttggagaccccgcgtgtccacagccgggcaccgtccccactctacagcgtggagttctctgaggagcccttcggggtgatcgtgcaccggcagctggacggccgcgtgctgctgaacacgacggtggcgcccctgttctttgcggaccagttccttcagctgtccacctcgctgccctcgcagtatatcacaggcctcgccgagcacctcagtcccctgatgctcagcaccagctggaccaggatcaccctgtggaaccgggaccttgcgcccacgcccggtgcgaacctctacgggtctcaccctttctacctggcgctggaggacggcgggtcggcacacggggtgttcctgctaaacagcaatgccatggatgtggtcctgcagccgagccctgcccttagctggaggtcgacaggtgggatcctggatgtctacatcttcctgggcccagagcccaagagcgtggtgcagcagtacctggacgttgtgggatacccgttcatgccgccatactggggcctgggcttccacctgtgccgctggggctactcctccaccgctatcacccgccaggtggtggagaacatgaccagggcccacttccccctggacgtccaatggaacgacctggactacatggactcccggagggacttcacgttcaacaaggatggcttccgggacttcccggccatggtgcaggagctgcaccagggcggccggcgctacatgatgatcgtggatcctgccatcagcagctcgggccctgccgggagctacaggccctacgacgagggtctgcggaggggggttttcatcaccaacgagaccggccagccgctgattgggaaggtatggcccgggtccactgccttccccgacttcaccaaccccacagccctggcctggtgggaggacatggtggctgagttccatgaccaggtgcccttcgacggcatgtggattgacatgaacgagccttccaacttcatcaggggctctgaggacggctgccccaacaatgagctggagaacccaccctacgtgcctggggtggttggggggaccctccaggcggcaaccatctgtgcctccagccaccagtttctctccacacactacaacctgcacaacctctacggcctgaccgaagccatcgcctcccacagggcgctggtgaaggctcgggggacacgcccatttgtgatctcccgctcgacctttgctggccacggccgatacgccggccactggacgggggacgtgtggagctcctgggagcagctcgcctcctccgtgccagaaatcctgcagtttaacctgctgggggtgcctctggtcggggccgacgtctgcggcttcctgggcaacacctcagaggagctgtgtgtgcgctggacccagctgggggccttctaccccttcatgcggaaccacaacagcctgctcagtctgccccaggagccgtacagcttcagcgagccggcccagcaggccatgaggaaggccctcaccctgcgctacgcactcctcccccacctctacacgctgttccaccaggcccacgtcgcgggggagaccgtggcccggcccctcttcctggagttccccaaggactctagcacctggactgtggaccaccagctcctgtggggggaggccctgctcatcaccccagtgctccaggccgggaaggccgaagtgactggctacttccccttgggcacatggtacgacctgcagacggtgccaatagaggcccttggcagcctcccacccccacctgcagctccccgtgagccagccatccacagcgaggggcagtgggtgacgctgccggcccccctggacaccatcaacgtccacctccgggctgggtacatcatccccctgcagggccctggcctcacaaccacagagtcccgccagcagcccatggccctggctgtggccctgaccaagggtggagaggcccgaggggagctgttctgggacgatggagagagcctggaagtgctggagcgaggggcctacacacaggtcatcttcctggccaggaataacacgatcgtgaatgagctggtacgtgtgaccagtgagggagctggcctgcagctgcagaaggtgactgtcctgggcgtggccacggcgccccagcaggtcctctccaacggtgtccctgtctccaacttcacctacagccccgacaccaaggtcctggacatctgtgtctcgctgttgatgggagagcagtttctcgtcagctggtgttagtctagagcttgctagcggccgc

SEQ ID NO: 24 - DNA, 2958 bp, Artificial Sequence
  GILTd2-7d36-39-GAA70-952 cassette
ggtaccagctgctagcaagctaattcacaccaatgggaatcccaatggggaagtcgatgctggtgcttctcaccttcttggccttcgcctcgtgctgcattgctgctctgtgcggcggggagctggtggacaccctccagttcgtctgtggggaccgcggcttctacttcagcaggcccgcaagccgtgtgcgtggcatcgttgaggagtgctgtttccgcagctgtgacctggccctcctggagacgtactgtgctacccccgccaagtccgagggcgcgccggcacaccccggccgtcccagagcagtgcccacacagtgcgacgtcccccccaacagccgcttcgattgcgcccctgacaaggccatcacccaggaacagtgcgaggcccgcggctgctgctacatccctgcaaagcaggggctgcagggagcccagatggggcagccctggtgcttcttcccacccagctaccccagctacaagctggagaacctgagctcctctgaaatgggctacacggccaccctgacccgtaccacccccaccttcttccccaaggacatcctgaccctgcggctggacgtgatgatggagactgagaaccgcctccacttcacgatcaaagatccagctaacaggcgctacgaggtgcccttggagaccccgcgtgtccacagccgggcaccgtccccactctacagcgtggagttctctgaggagcccttcggggtgatcgtgcaccggcagctggacggccgcgtgctgctgaacacgacggtggcgcccctgttctttgcggaccagttccttcagctgtccacctcgctgccctcgcagtatatcacaggcctcgccgagcacctcagtcccctgatgctcagcaccagctggaccaggatcaccctgtggaaccgggaccttgcgcccacgcccggtgcgaacctctacgggtctcaccctttctacctggcgctggaggacggcgggtcggcacacggggtgttcctgctaaacagcaatgccatggatgtggtcctgcagccgagccctgcccttagctggaggtcgacaggtgggatcctggatgtctacatcttcctgggcccagagcccaagagcgtggtgcagcagtacctggacgttgtgggatacccgttcatgccgccatactggggcctgggcttccacctgtgccgctggggctactcctccaccgctatcacccgccaggtggtggagaacatgaccagggcccacttccccctggacgtccaatggaacgacctggactacatggactcccggagggacttcacgttcaacaaggatggcttccgggacttcccggccatggtgcaggagctgcaccagggcggccggcgctacatgatgatcgtggatcctgccatcagcagctcgggccctgccgggagctacaggccctacgacgagggtctgcggaggggggttttcatcaccaacgagaccggccagccgctgattgggaaggtatggcccgggtccactgccttccccgacttcaccaaccccacagccctggcctggtgggaggacatggtggctgagttccatgaccaggtgcccttcgacggcatgtggattgacatgaacgagccttccaacttcatcaggggctctgaggacggctgccccaacaatgagctggagaacccaccctacgtgcctggggtggttggggggaccctccaggcggcaaccatctgtgcctccagccaccagtttctctccacacactacaacctgcacaacctctacggcctgaccgaagccatcgcctcccacagggcgctggtgaaggctcgggggacacgcccatttgtgatctcccgctcgacctttgctggccacggccgatacgccggccactggacgggggacgtgtggagctcctgggagcagctcgcctcctccgtgccagaaatcctgcagtttaacctgctgggggtgcctctggtcggggccgacgtctgcggcttcctgggcaacacctcagaggagctgtgtgtgcgctggacccagctgggggccttctaccccttcatgcggaaccacaacagcctgctcagtctgccccaggagccgtacagcttcagcgagccggcccagcaggccatgaggaaggccctcaccctgcgctacgcactcctcccccacctctacacgctgttccaccaggcccacgtcgcgggggagaccgtggcccggcccctcttcctggagttccccaaggactctagcacctggactgtggaccaccagctcctgtggggggaggccctgctcatcaccccagtgctccaggccgggaaggccgaagtgactggctacttccccttgggcacatggtacgacctgcagacggtgccaatagaggcccttggcagcctcccacccccacctgcagctccccgtgagccagccatccacagcgaggggcagtgggtgacgctgccggcccccctggacaccatcaacgtccacctccgggctgggtacatcatccccctgcagggccctggcctcacaaccacagagtcccgccagcagcccatggccctggctgtggccctgaccaagggtggagaggcccgaggggagctgttctgggacgatggagagagcctggaagtgctggagcgaggggcctacacacaggtcatcttcctggccaggaataacacgatcgtgaatgagctggtacgtgtgaccagtgagggagctggcctgcagctgcagaaggtgactgtcctgggcgtggccacggcgccccagcaggtcctctccaacggtgtccctgtctccaacttcacctacagccccgacaccaaggtcctggacatctgtgtctcgctgttgatgggagagcagtttctcgtcagctggtgttagtctagagcttgctagcggccgc

SEQ ID NO: 25 - DNA, 2934 bp, Artificial Sequence
  GILTd2-7d29-40-GAA70-952 cassette
ggtaccagctgctagcaagctaattcacaccaatgggaatcccaatggggaagtcgatgctggtgcttctcaccttcttggccttcgcctcgtgctgcattgctgctctgtgcggcggggagctggtggacaccctccagttcgtctgtggggaccgcggcttctacttcggcatcgttgaggagtgctgtttccgcagctgtgacctggccctcctggagacgtactgtgctacccccgccaagtccgagggcgcgccggcacaccccggccgtcccagagcagtgcccacacagtgcgacgtcccccccaacagccgcttcgattgcgcccctgacaaggccatcacccaggaacagtgcgaggcccgcggctgctgctacatccctgcaaagcaggggctgcagggagcccagatggggcagccctggtgcttcttcccacccagctaccccagctacaagctggagaacctgagctcctctgaaatgggctacacggccaccctgacccgtaccacccccaccttcttccccaaggacatcctgaccctgcggctggacgtgatgatggagactgagaaccgcctccacttcacgatcaaagatccagctaacaggcgctacgaggtgcccttggagaccccgcgtgtccacagccgggcaccgtccccactctacagcgtggagttctctgaggagcccttcggggtgatcgtgcaccggcagctggacggccgcgtgctgctgaacacgacggtggcgcccctgttctttgcggaccagttccttcagctgtccacctcgctgccctcgcagtatatcacaggcctcgccgagcacctcagtcccctgatgctcagcaccagctggaccaggatcaccctgtggaaccgggaccttgcgcccacgcccggtgcgaacctctacgggtctcaccctttctacctggcgctggaggacggcgggtcggcacacggggtgttcctgctaaacagcaatgccatggatgtggtcctgcagccgagccctgcccttagctggaggtcgacaggtgggatcctggatgtctacatcttcctgggcccagagcccaagagcgtggtgcagcagtacctggacgttgtgggatacccgttcatgccgccatactggggcctgggcttccacctgtgccgctggggctactcctccaccgctatcacccgccaggtggtggagaacatgaccagggcccacttccccctggacgtccaatggaacgacctggactacatggactcccggagggacttcacgttcaacaaggatggcttccgggacttcccggccatggtgcaggagctgcaccagggcggccggcgctacatgatgatcgtggatcctgccatcagcagctcgggccctgccgggagctacaggccctacgacgagggtctgcggaggggggttttcatcaccaacgagaccggccagccgctgattgggaaggtatggcccgggtccactgccttccccgacttcaccaaccccacagccctggcctggtgggaggacatggtggctgagttccatgaccaggtgcccttcgacggcatgtggattgacatgaacgagccttccaacttcatcaggggctctgaggacggctgccccaacaatgagctggagaacccaccctacgtgcctggggtggttggggggaccctccaggcggcaaccatctgtgcctccagccaccagtttctctccacacactacaacctgcacaacctctacggcctgaccgaagccatcgcctcccacagggcgctggtgaaggctcgggggacacgcccatttgtgatctcccgctcgacctttgctggccacggccgatacgccggccactggacgggggacgtgtggagctcctgggagcagctcgcctcctccgtgccagaaatcctgcagtttaacctgctgggggtgcctctggtcggggccgacgtctgcggcttcctgggcaacacctcagaggagctgtgtgtgcgctggacccagctgggggccttctaccccttcatgcggaaccacaacagcctgctcagtctgccccaggagccgtacagcttcagcgagccggcccagcaggccatgaggaaggccctcaccctgcgctacgcactcctcccccacctctacacgctgttccaccaggcccacgtcgcgggggagaccgtggcccggcccctcttcctggagttccccaaggactctagcacctggactgtggaccaccagctcctgtggggggaggccctgctcatcaccccagtgctccaggccgggaaggccgaagtgactggctacttccccttgggcacatggtacgacctgcagacggtgccaatagaggcccttggcagcctcccacccccacctgcagctccccgtgagccagccatccacagcgaggggcagtgggtgacgctgccggcccccctggacaccatcaacgtccacctccgggctgggtacatcatccccctgcagggccctggcctcacaaccacagagtcccgccagcagcccatggccctggctgtggccctgaccaagggtggagaggcccgaggggagctgttctgggacgatggagagagcctggaagtgctggagcgaggggcctacacacaggtcatcttcctggccaggaataacacgatcgtgaatgagctggtacgtgtgaccagtgagggagctggcctgcagctgcagaaggtgactgtcctgggcgtggccacggcgccccagcaggtcctctccaacggtgtccctgtctccaacttcacctacagccccgacaccaaggtcctggacatctgtgtctcgctgttgatgggagagcagtttctcgtcagctggtgttagtctagagcttgctagcggccgc

SEQ ID NO: 26 - DNA, 2937 bp, Artificial Sequence
  GILTd2-7d30-40-GAA70-952 cassette
ggtaccagctgctagcaagctaattcacaccaatgggaatcccaatggggaagtcgatgctggtgcttctcaccttcttggccttcgcctcgtgctgcattgctgctctgtgcggcggggagctggtggacaccctccagttcgtctgtggggaccgcggcttctacttcagcggcatcgttgaggagtgctgtttccgcagctgtgacctggccctcctggagacgtactgtgctacccccgccaagtccgagggcgcgccggcacaccccggccgtcccagagcagtgcccacacagtgcgacgtcccccccaacagccgcttcgattgcgcccctgacaaggccatcacccaggaacagtgcgaggcccgcggctgctgctacatccctgcaaagcaggggctgcagggagcccagatggggcagccctggtgcttcttcccacccagctaccccagctacaagctggagaacctgagctcctctgaaatgggctacacggccaccctgacccgtaccacccccaccttcttccccaaggacatcctgaccctgcggctggacgtgatgatggagactgagaaccgcctccacttcacgatcaaagatccagctaacaggcgctacgaggtgcccttggagaccccgcgtgtccacagccgggcaccgtccccactctacagcgtggagttctctgaggagcccttcggggtgatcgtgcaccggcagctggacggccgcgtgctgctgaacacgacggtggcgcccctgttctttgcggaccagttccttcagctgtccacctcgctgccctcgcagtatatcacaggcctcgccgagcacctcagtcccctgatgctcagcaccagctggaccaggatcaccctgtggaaccgggaccttgcgcccacgcccggtgcgaacctctacgggtctcaccctttctacctggcgctggaggacggcgggtcggcacacggggtgttcctgctaaacagcaatgccatggatgtggtcctgcagccgagccctgcccttagctggaggtcgacaggtgggatcctggatgtctacatcttcctgggcccagagcccaagagcgtggtgcagcagtacctggacgttgtgggatacccgttcatgccgccatactggggcctgggcttccacctgtgccgctggggctactcctccaccgctatcacccgccaggtggtggagaacatgaccagggcccacttccccctggacgtccaatggaacgacctggactacatggactcccggagggacttcacgttcaacaaggatggcttccgggacttcccggccatggtgcaggagctgcaccagggcggccggcgctacatgatgatcgtggatcctgccatcagcagctcgggccctgccgggagctacaggccctacgacgagggtctgcggaggggggttttcatcaccaacgagaccggccagccgctgattgggaaggtatggcccgggtccactgccttccccgacttcaccaaccccacagccctggcctggtgggaggacatggtggctgagttccatgaccaggtgcccttcgacggcatgtggattgacatgaacgagccttccaacttcatcaggggctctgaggacggctgccccaacaatgagctggagaacccaccctacgtgcctggggtggttggggggaccctccaggcggcaaccatctgtgcctccagccaccagtttctctccacacactacaacctgcacaacctctacggcctgaccgaagccatcgcctcccacagggcgctggtgaaggctcgggggacacgcccatttgtgatctcccgctcgacctttgctggccacggccgatacgccggccactggacgggggacgtgtggagctcctgggagcagctcgcctcctccgtgccagaaatcctgcagtttaacctgctgggggtgcctctggtcggggccgacgtctgcggcttcctgggcaacacctcagaggagctgtgtgtgcgctggacccagctgggggccttctaccccttcatgcggaaccacaacagcctgctcagtctgccccaggagccgtacagcttcagcgagccggcccagcaggccatgaggaaggccctcaccctgcgctacgcactcctcccccacctctacacgctgttccaccaggcccacgtcgcgggggagaccgtggcccggcccctcttcctggagttccccaaggactctagcacctggactgtggaccaccagctcctgtggggggaggccctgctcatcaccccagtgctccaggccgggaaggccgaagtgactggctacttccccttgggcacatggtacgacctgcagacggtgccaatagaggcccttggcagcctcccacccccacctgcagctccccgtgagccagccatccacagcgaggggcagtgggtgacgctgccggcccccctggacaccatcaacgtccacctccgggctgggtacatcatccccctgcagggccctggcctcacaaccacagagtcccgccagcagcccatggccctggctgtggccctgaccaagggtggagaggcccgaggggagctgttctgggacgatggagagagcctggaagtgctggagcgaggggcctacacacaggtcatcttcctggccaggaataacacgatcgtgaatgagctggtacgtgtgaccagtgagggagctggcctgcagctgcagaaggtgactgtcctgggcgtggccacggcgccccagcaggtcctctccaacggtgtccctgtctccaacttcacctacagccccgacaccaaggtcctggacatctgtgtctcgctgttgatgggagagcagtttctcgtcagctggtgttagtctagagcttgctagcggccgc

SEQ ID NO: 27 - DNA, 2940 bp, Artificial Sequence
  GILTd2-7d31-40-GAA70-952 cassette
ggtaccagctgctagcaagctaattcacaccaatgggaatcccaatggggaagtcgatgctggtgcttctcaccttcttggccttcgcctcgtgctgcattgctgctctgtgcggcggggagctggtggacaccctccagttcgtctgtggggaccgcggcttctacttcagcaggggcatcgttgaggagtgctgtttccgcagctgtgacctggccctcctggagacgtactgtgctacccccgccaagtccgagggcgcgccggcacaccccggccgtcccagagcagtgcccacacagtgcgacgtcccccccaacagccgcttcgattgcgcccctgacaaggccatcacccaggaacagtgcgaggcccgcggctgctgctacatccctgcaaagcaggggctgcagggagcccagatggggcagccctggtgcttcttcccacccagctaccccagctacaagctggagaacctgagctcctctgaaatgggctacacggccaccctgacccgtaccacccccaccttcttccccaaggacatcctgaccctgcggctggacgtgatgatggagactgagaaccgcctccacttcacgatcaaagatccagctaacaggcgctacgaggtgcccttggagaccccgcgtgtccacagccgggcaccgtccccactctacagcgtggagttctctgaggagcccttcggggtgatcgtgcaccggcagctggacggccgcgtgctgctgaacacgacggtggcgcccctgttctttgcggaccagttccttcagctgtccacctcgctgccctcgcagtatatcacaggcctcgccgagcacctcagtcccctgatgctcagcaccagctggaccaggatcaccctgtggaaccgggaccttgcgcccacgcccggtgcgaacctctacgggtctcaccctttctacctggcgctggaggacggcgggtcggcacacggggtgttcctgctaaacagcaatgccatggatgtggtcctgcagccgagccctgcccttagctggaggtcgacaggtgggatcctggatgtctacatcttcctgggcccagagcccaagagcgtggtgcagcagtacctggacgttgtgggatacccgttcatgccgccatactggggcctgggcttccacctgtgccgctggggctactcctccaccgctatcacccgccaggtggtggagaacatgaccagggcccacttccccctggacgtccaatggaacgacctggactacatggactcccggagggacttcacgttcaacaaggatggcttccgggacttcccggccatggtgcaggagctgcaccagggcggccggcgctacatgatgatcgtggatcctgccatcagcagctcgggccctgccgggagctacaggccctacgacgagggtctgcggaggggggttttcatcaccaacgagaccggccagccgctgattgggaaggtatggcccgggtccactgccttccccgacttcaccaaccccacagccctggcctggtgggaggacatggtggctgagttccatgaccaggtgcccttcgacggcatgtggattgacatgaacgagccttccaacttcatcaggggctctgaggacggctgccccaacaatgagctggagaacccaccctacgtgcctggggtggttggggggaccctccaggcggcaaccatctgtgcctccagccaccagtttctctccacacactacaacctgcacaacctctacggcctgaccgaagccatcgcctcccacagggcgctggtgaaggctcgggggacacgcccatttgtgatctcccgctcgacctttgctggccacggccgatacgccggccactggacgggggacgtgtggagctcctgggagcagctcgcctcctccgtgccagaaatcctgcagtttaacctgctgggggtgcctctggtcggggccgacgtctgcggcttcctgggcaacacctcagaggagctgtgtgtgcgctggacccagctgggggccttctaccccttcatgcggaaccacaacagcctgctcagtctgccccaggagccgtacagcttcagcgagccggcccagcaggccatgaggaaggccctcaccctgcgctacgcactcctcccccacctctacacgctgttccaccaggcccacgtcgcgggggagaccgtggcccggcccctcttcctggagttccccaaggactctagcacctggactgtggaccaccagctcctgtggggggaggccctgctcatcaccccagtgctccaggccgggaaggccgaagtgactggctacttccccttgggcacatggtacgacctgcagacggtgccaatagaggcccttggcagcctcccacccccacctgcagctccccgtgagccagccatccacagcgaggggcagtgggtgacgctgccggcccccctggacaccatcaacgtccacctccgggctgggtacatcatccccctgcagggccctggcctcacaaccacagagtcccgccagcagcccatggccctggctgtggccctgaccaagggtggagaggcccgaggggagctgttctgggacgatggagagagcctggaagtgctggagcgaggggcctacacacaggtcatcttcctggccaggaataacacgatcgtgaatgagctggtacgtgtgaccagtgagggagctggcctgcagctgcagaaggtgactgtcctgggcgtggccacggcgccccagcaggtcctctccaacggtgtccctgtctccaacttcacctacagccccgacaccaaggtcctggacatctgtgtctcgctgttgatgggagagcagtttctcgtcagctggtgttagtctagagcttgctagcggccgc

SEQ ID NO: 28 - DNA, 2943 bp, Artificial Sequence
  GILTd2-7d32-40-GAA70-952 cassette
ggtaccagctgctagcaagctaattcacaccaatgggaatcccaatggggaagtcgatgctggtgcttctcaccttcttggccttcgcctcgtgctgcattgctgctctgtgcggcggggagctggtggacaccctccagttcgtctgtggggaccgcggcttctacttcagcaggcccggcatcgttgaggagtgctgtttccgcagctgtgacctggccctcctggagacgtactgtgctacccccgccaagtccgagggcgcgccggcacaccccggccgtcccagagcagtgcccacacagtgcgacgtcccccccaacagccgcttcgattgcgcccctgacaaggccatcacccaggaacagtgcgaggcccgcggctgctgctacatccctgcaaagcaggggctgcagggagcccagatggggcagccctggtgcttcttcccacccagctaccccagctacaagctggagaacctgagctcctctgaaatgggctacacggccaccctgacccgtaccacccccaccttcttccccaaggacatcctgaccctgcggctggacgtgatgatggagactgagaaccgcctccacttcacgatcaaagatccagctaacaggcgctacgaggtgcccttggagaccccgcgtgtccacagccgggcaccgtccccactctacagcgtggagttctctgaggagcccttcggggtgatcgtgcaccggcagctggacggccgcgtgctgctgaacacgacggtggcgcccctgttctttgcggaccagttccttcagctgtccacctcgctgccctcgcagtatatcacaggcctcgccgagcacctcagtcccctgatgctcagcaccagctggaccaggatcaccctgtggaaccgggaccttgcgcccacgcccggtgcgaacctctacgggtctcaccctttctacctggcgctggaggacggcgggtcggcacacggggtgttcctgctaaacagcaatgccatggatgtggtcctgcagccgagccctgcccttagctggaggtcgacaggtgggatcctggatgtctacatcttcctgggcccagagcccaagagcgtggtgcagcagtacctggacgttgtgggatacccgttcatgccgccatactggggcctgggcttccacctgtgccgctggggctactcctccaccgctatcacccgccaggtggtggagaacatgaccagggcccacttccccctggacgtccaatggaacgacctggactacatggactcccggagggacttcacgttcaacaaggatggcttccgggacttcccggccatggtgcaggagctgcaccagggcggccggcgctacatgatgatcgtggatcctgccatcagcagctcgggccctgccgggagctacaggccctacgacgagggtctgcggaggggggttttcatcaccaacgagaccggccagccgctgattgggaaggtatggcccgggtccactgccttccccgacttcaccaaccccacagccctggcctggtgggaggacatggtggctgagttccatgaccaggtgcccttcgacggcatgtggattgacatgaacgagccttccaacttcatcaggggctctgaggacggctgccccaacaatgagctggagaacccaccctacgtgcctggggtggttggggggaccctccaggcggcaaccatctgtgcctccagccaccagtttctctccacacactacaacctgcacaacctctacggcctgaccgaagccatcgcctcccacagggcgctggtgaaggctcgggggacacgcccatttgtgatctcccgctcgacctttgctggccacggccgatacgccggccactggacgggggacgtgtggagctcctgggagcagctcgcctcctccgtgccagaaatcctgcagtttaacctgctgggggtgcctctggtcggggccgacgtctgcggcttcctgggcaacacctcagaggagctgtgtgtgcgctggacccagctgggggccttctaccccttcatgcggaaccacaacagcctgctcagtctgccccaggagccgtacagcttcagcgagccggcccagcaggccatgaggaaggccctcaccctgcgctacgcactcctcccccacctctacacgctgttccaccaggcccacgtcgcgggggagaccgtggcccggcccctcttcctggagttccccaaggactctagcacctggactgtggaccaccagctcctgtggggggaggccctgctcatcaccccagtgctccaggccgggaaggccgaagtgactggctacttccccttgggcacatggtacgacctgcagacggtgccaatagaggcccttggcagcctcccacccccacctgcagctccccgtgagccagccatccacagcgaggggcagtgggtgacgctgccggcccccctggacaccatcaacgtccacctccgggctgggtacatcatccccctgcagggccctggcctcacaaccacagagtcccgccagcagcccatggccctggctgtggccctgaccaagggtggagaggcccgaggggagctgttctgggacgatggagagagcctggaagtgctggagcgaggggcctacacacaggtcatcttcctggccaggaataacacgatcgtgaatgagctggtacgtgtgaccagtgagggagctggcctgcagctgcagaaggtgactgtcctgggcgtggccacggcgccccagcaggtcctctccaacggtgtccctgtctccaacttcacctacagccccgacaccaaggtcctggacatctgtgtctcgctgttgatgggagagcagtttctcgtcagctggtgttagtctagagcttgctagcggccgc

SEQ ID NO: 29 - DNA, 2946 bp, Artificial Sequence
  GILTd2-7d33-40-GAA70-952 cassette
ggtaccagctgctagcaagctaattcacaccaatgggaatcccaatggggaagtcgatgctggtgcttctcaccttcttggccttcgcctcgtgctgcattgctgctctgtgcggcggggagctggtggacaccctccagttcgtctgtggggaccgcggcttctacttcagcaggcccgcaggcatcgttgaggagtgctgtttccgcagctgtgacctggccctcctggagacgtactgtgctacccccgccaagtccgagggcgcgccggcacaccccggccgtcccagagcagtgcccacacagtgcgacgtcccccccaacagccgcttcgattgcgcccctgacaaggccatcacccaggaacagtgcgaggcccgcggctgctgctacatccctgcaaagcaggggctgcagggagcccagatggggcagccctggtgcttcttcccacccagctaccccagctacaagctggagaacctgagctcctctgaaatgggctacacggccaccctgacccgtaccacccccaccttcttccccaaggacatcctgaccctgcggctggacgtgatgatggagactgagaaccgcctccacttcacgatcaaagatccagctaacaggcgctacgaggtgcccttggagaccccgcgtgtccacagccgggcaccgtccccactctacagcgtggagttctctgaggagcccttcggggtgatcgtgcaccggcagctggacggccgcgtgctgctgaacacgacggtggcgcccctgttctttgcggaccagttccttcagctgtccacctcgctgccctcgcagtatatcacaggcctcgccgagcacctcagtcccctgatgctcagcaccagctggaccaggatcaccctgtggaaccgggaccttgcgcccacgcccggtgcgaacctctacgggtctcaccctttctacctggcgctggaggacggcgggtcggcacacggggtgttcctgctaaacagcaatgccatggatgtggtcctgcagccgagccctgcccttagctggaggtcgacaggtgggatcctggatgtctacatcttcctgggcccagagcccaagagcgtggtgcagcagtacctggacgttgtgggatacccgttcatgccgccatactggggcctgggcttccacctgtgccgctggggctactcctccaccgctatcacccgccaggtggtggagaacatgaccagggcccacttccccctggacgtccaatggaacgacctggactacatggactcccggagggacttcacgttcaacaaggatggcttccgggacttcccggccatggtgcaggagctgcaccagggcggccggcgctacatgatgatcgtggatcctgccatcagcagctcgggccctgccgggagctacaggccctacgacgagggtctgcggaggggggttttcatcaccaacgagaccggccagccgctgattgggaaggtatggcccgggtccactgccttccccgacttcaccaaccccacagccctggcctggtgggaggacatggtggctgagttccatgaccaggtgcccttcgacggcatgtggattgacatgaacgagccttccaacttcatcaggggctctgaggacggctgccccaacaatgagctggagaacccaccctacgtgcctggggtggttggggggaccctccaggcggcaaccatctgtgcctccagccaccagtttctctccacacactacaacctgcacaacctctacggcctgaccgaagccatcgcctcccacagggcgctggtgaaggctcgggggacacgcccatttgtgatctcccgctcgacctttgctggccacggccgatacgccggccactggacgggggacgtgtggagctcctgggagcagctcgcctcctccgtgccagaaatcctgcagtttaacctgctgggggtgcctctggtcggggccgacgtctgcggcttcctgggcaacacctcagaggagctgtgtgtgcgctggacccagctgggggccttctaccccttcatgcggaaccacaacagcctgctcagtctgccccaggagccgtacagcttcagcgagccggcccagcaggccatgaggaaggccctcaccctgcgctacgcactcctcccccacctctacacgctgttccaccaggcccacgtcgcgggggagaccgtggcccggcccctcttcctggagttccccaaggactctagcacctggactgtggaccaccagctcctgtggggggaggccctgctcatcaccccagtgctccaggccgggaaggccgaagtgactggctacttccccttgggcacatggtacgacctgcagacggtgccaatagaggcccttggcagcctcccacccccacctgcagctccccgtgagccagccatccacagcgaggggcagtgggtgacgctgccggcccccctggacaccatcaacgtccacctccgggctgggtacatcatccccctgcagggccctggcctcacaaccacagagtcccgccagcagcccatggccctggctgtggccctgaccaagggtggagaggcccgaggggagctgttctgggacgatggagagagcctggaagtgctggagcgaggggcctacacacaggtcatcttcctggccaggaataacacgatcgtgaatgagctggtacgtgtgaccagtgagggagctggcctgcagctgcagaaggtgactgtcctgggcgtggccacggcgccccagcaggtcctctccaacggtgtccctgtctccaacttcacctacagccccgacaccaaggtcctggacatctgtgtctcgctgttgatgggagagcagtttctcgtcagctggtgttagtctagagcttgctagcggccgc

SEQ ID NO: 30 - DNA, 2949 bp, Artificial Sequence
  GILTd2-7d34-40-GAA70-952 cassette
ggtaccagctgctagcaagctaattcacaccaatgggaatcccaatggggaagtcgatgctggtgcttctcaccttcttggccttcgcctcgtgctgcattgctgctctgtgcggcggggagctggtggacaccctccagttcgtctgtggggaccgcggcttctacttcagcaggcccgcaagcggcatcgttgaggagtgctgtttccgcagctgtgacctggccctcctggagacgtactgtgctacccccgccaagtccgagggcgcgccggcacaccccggccgtcccagagcagtgcccacacagtgcgacgtcccccccaacagccgcttcgattgcgcccctgacaaggccatcacccaggaacagtgcgaggcccgcggctgctgctacatccctgcaaagcaggggctgcagggagcccagatggggcagccctggtgcttcttcccacccagctaccccagctacaagctggagaacctgagctcctctgaaatgggctacacggccaccctgacccgtaccacccccaccttcttccccaaggacatcctgaccctgcggctggacgtgatgatggagactgagaaccgcctccacttcacgatcaaagatccagctaacaggcgctacgaggtgcccttggagaccccgcgtgtccacagccgggcaccgtccccactctacagcgtggagttctctgaggagcccttcggggtgatcgtgcaccggcagctggacggccgcgtgctgctgaacacgacggtggcgcccctgttctttgcggaccagttccttcagctgtccacctcgctgccctcgcagtatatcacaggcctcgccgagcacctcagtcccctgatgctcagcaccagctggaccaggatcaccctgtggaaccgggaccttgcgcccacgcccggtgcgaacctctacgggtctcaccctttctacctggcgctggaggacggcgggtcggcacacggggtgttcctgctaaacagcaatgccatggatgtggtcctgcagccgagccctgcccttagctggaggtcgacaggtgggatcctggatgtctacatcttcctgggcccagagcccaagagcgtggtgcagcagtacctggacgttgtgggatacccgttcatgccgccatactggggcctgggcttccacctgtgccgctggggctactcctccaccgctatcacccgccaggtggtggagaacatgaccagggcccacttccccctggacgtccaatggaacgacctggactacatggactcccggagggacttcacgttcaacaaggatggcttccgggacttcccggccatggtgcaggagctgcaccagggcggccggcgctacatgatgatcgtggatcctgccatcagcagctcgggccctgccgggagctacaggccctacgacgagggtctgcggaggggggttttcatcaccaacgagaccggccagccgctgattgggaaggtatggcccgggtccactgccttccccgacttcaccaaccccacagccctggcctggtgggaggacatggtggctgagttccatgaccaggtgcccttcgacggcatgtggattgacatgaacgagccttccaacttcatcaggggctctgaggacggctgccccaacaatgagctggagaacccaccctacgtgcctggggtggttggggggaccctccaggcggcaaccatctgtgcctccagccaccagtttctctccacacactacaacctgcacaacctctacggcctgaccgaagccatcgcctcccacagggcgctggtgaaggctcgggggacacgcccatttgtgatctcccgctcgacctttgctggccacggccgatacgccggccactggacgggggacgtgtggagctcctgggagcagctcgcctcctccgtgccagaaatcctgcagtttaacctgctgggggtgcctctggtcggggccgacgtctgcggcttcctgggcaacacctcagaggagctgtgtgtgcgctggacccagctgggggccttctaccccttcatgcggaaccacaacagcctgctcagtctgccccaggagccgtacagcttcagcgagccggcccagcaggccatgaggaaggccctcaccctgcgctacgcactcctcccccacctctacacgctgttccaccaggcccacgtcgcgggggagaccgtggcccggcccctcttcctggagttccccaaggactctagcacctggactgtggaccaccagctcctgtggggggaggccctgctcatcaccccagtgctccaggccgggaaggccgaagtgactggctacttccccttgggcacatggtacgacctgcagacggtgccaatagaggcccttggcagcctcccacccccacctgcagctccccgtgagccagccatccacagcgaggggcagtgggtgacgctgccggcccccctggacaccatcaacgtccacctccgggctgggtacatcatccccctgcagggccctggcctcacaaccacagagtcccgccagcagcccatggccctggctgtggccctgaccaagggtggagaggcccgaggggagctgttctgggacgatggagagagcctggaagtgctggagcgaggggcctacacacaggtcatcttcctggccaggaataacacgatcgtgaatgagctggtacgtgtgaccagtgagggagctggcctgcagctgcagaaggtgactgtcctgggcgtggccacggcgccccagcaggtcctctccaacggtgtccctgtctccaacttcacctacagccccgacaccaaggtcctggacatctgtgtctcgctgttgatgggagagcagtttctcgtcagctggtgttagtctagagcttgctagcggccgc

SEQ ID NO: 31 - DNA, 2953 bp, Artificial Sequence
  GILTd2-7M1/L27A37-GAA70-952 cassette
ggtaccaagcttgccatgggaatcccaatgggcaagtcgatgctggtgctgctcaccttcttggcctttgcctcgtgctgcattgccgctctgtgcggcggggaactggtggacaccctccaattcgtctgtggggaccggggcttcctgttcagcagacccgcaagccgtgtgagtgctcgcagccgtggcattgttgaggagtgctgttttcgcagctgtgacctggctctcctggagacgtactgcgctacccccgccaagtctgagggcgcgccggcacaccccggccgtcccagagcagtgcccacacagtgcgacgtcccccccaacagccgcttcgattgcgcccctgacaaggccatcacccaggaacagtgcgaggcccgcggctgctgctacatccctgcaaagcaggggctgcagggagcccagatggggcagccctggtgcttcttcccacccagctaccccagctacaagctggagaacctgagctcctctgaaatgggctacacggccaccctgacccgtaccacccccaccttcttccccaaggacatcctgaccctgcggctggacgtgatgatggagactgagaaccgcctccacttcacgatcaaagatccagctaacaggcgctacgaggtgcccttggagaccccgcgtgtccacagccgggcaccgtccccactctacagcgtggagttctctgaggagcccttcggggtgatcgtgcaccggcagctggacggccgcgtgctgctgaacacgacggtggcgcccctgttctttgcggaccagttccttcagctgtccacctcgctgccctcgcagtatatcacaggcctcgccgagcacctcagtcccctgatgctcagcaccagctggaccaggatcaccctgtggaaccgggaccttgcgcccacgcccggtgcgaacctctacgggtctcaccctttctacctggcgctggaggacggcgggtcggcacacggggtgttcctgctaaacagcaatgccatggatgtggtcctgcagccgagccctgcccttagctggaggtcgacaggtgggatcctggatgtctacatcttcctgggcccagagcccaagagcgtggtgcagcagtacctggacgttgtgggatacccgttcatgccgccatactggggcctgggcttccacctgtgccgctggggctactcctccaccgctatcacccgccaggtggtggagaacatgaccagggcccacttccccctggacgtccaatggaacgacctggactacatggactcccggagggacttcacgttcaacaaggatggcttccgggacttcccggccatggtgcaggagctgcaccagggcggccggcgctacatgatgatcgtggatcctgccatcagcagctcgggccctgccgggagctacaggccctacgacgagggtctgcggaggggggttttcatcaccaacgagaccggccagccgctgattgggaaggtatggcccgggtccactgccttccccgacttcaccaaccccacagccctggcctggtgggaggacatggtggctgagttccatgaccaggtgcccttcgacggcatgtggattgacatgaacgagccttccaacttcatcaggggctctgaggacggctgccccaacaatgagctggagaacccaccctacgtgcctggggtggttggggggaccctccaggcggcaaccatctgtgcctccagccaccagtttctctccacacactacaacctgcacaacctctacggcctgaccgaagccatcgcctcccacagggcgctggtgaaggctcgggggacacgcccatttgtgatctcccgctcgacctttgctggccacggccgatacgccggccactggacgggggacgtgtggagctcctgggagcagctcgcctcctccgtgccagaaatcctgcagtttaacctgctgggggtgcctctggtcggggccgacgtctgcggcttcctgggcaacacctcagaggagctgtgtgtgcgctggacccagctgggggccttctaccccttcatgcggaaccacaacagcctgctcagtctgccccaggagccgtacagcttcagcgagccggcccagcaggccatgaggaaggccctcaccctgcgctacgcactcctcccccacctctacacgctgttccaccaggcccacgtcgcgggggagaccgtggcccggcccctcttcctggagttccccaaggactctagcacctggactgtggaccaccagctcctgtggggggaggccctgctcatcaccccagtgctccaggccgggaaggccgaagtgactggctacttccccttgggcacatggtacgacctgcagacggtgccaatagaggcccttggcagcctcccacccccacctgcagctccccgtgagccagccatccacagcgaggggcagtgggtgacgctgccggcccccctggacaccatcaacgtccacctccgggctgggtacatcatccccctgcagggccctggcctcacaaccacagagtcccgccagcagcccatggccctggctgtggccctgaccaagggtggagaggcccgaggggagctgttctgggacgatggagagagcctggaagtgctggagcgaggggcctacacacaggtcatcttcctggccaggaataacacgatcgtgaatgagctggtacgtgtgaccagtgagggagctggcctgcagctgcagaaggtgactgtcctgggcgtggccacggcgccccagcaggtcctctccaacggtgtccctgtctccaacttcacctacagccccgacaccaaggtcctggacatctgtgtctcgctgttgatgggagagcagtttctcgtcagctggtgttagtctagagcttgctagcggccgc

SEQ ID NO: 32 - protein, 8 aa, Artificial Sequence
  Furin cleavage site - ZC-701
RVSRRSRG

SEQ ID NO: 33 - protein, 8 aa, Artificial Sequence
  Furin cleavage site - p1459 K37
RVSKRSRG

SEQ ID NO: 34 - protein, 8 aa, Artificial Sequence
  Furin cleavage site - p1460 K40
RVSRRSKG

SEQ ID NO: 35 - protein, 8 aa, Artificial Sequence
  Furin cleavage site - p1461 A37
RVSARSRG